European Patent Application EP 4 756 026 A1, published June 10, 2026. Title: 基因编辑系统及其应用. Applicant: 广州瑞风生物科技有限公司. Application WO. The sequence listing filed with the application follows.

SEQUENCE LISTING (410 sequences)

SEQ ID NO: 1 - protein, 893 aa, synthetic construct
MSKDKKTKAKRMGVKALLAHGEDKLTMTTFGKGNRSKIEFTEGYHGRALETPKHFGIRGFEVRRIDENVDLCGDLEEGKTIEALLVNPSEKVGEDYLKLKGTLEKRFFGREFPHDNIRIQLIYNILDIYKILGMNVADILYALGNMQDTELDIDMFGQSLNNEDNLKECLKRMRPYMGYFGDIFKISPKGENIADREHNKKVLRCISVLRNATAHDKQDEYPWFKSSDIYETKIFKADMWKIIKDQYREKIKKVNKDFLSKNAVNMAILFDLLNARDVEQKKQITDEFYRFTIRKDGKNLGMNLVKIREIIIDRYASGLRDKKHDPHRQKINVIADFLIFRALSQNQGIIDKTVSSLRLTKDEEEKDHVYQNAAELVWGMVSNCLTPYFNDPKNKYILKYKDAKTPGDFEDWITSKISEDDGEPFVKVLSFLCNFLEGKEINELLTAYIHKFECIQDFLNVISSLGENVQFQPRFALFNNASFAQNVAVQLRILASIGKMKPDLTEAKRPLYKAAIRMLCPPEKWEKYTSDEWLEKNMLLNSEDRKNDKKKKQVNPFRNFIAGNVIESRRFMYLVRYSKPKAVRAIMQNRSIVNYVLHRLPSEQVHRYASVFPENFADLEQEIDFLTKKLFEFSFEELLHEKDVILNNSRSHKPSLEIERLKAITGLYLSVAYIAIKNIVKANARYYIAFAVFERDKELVKAKDARIQTKIPETDFPDYFCLTQYYLDRDEEKKFPGDPRDKEAFFEHLRKTKRHFSKQWREWLNEKIADAKSSQATGLLLREARNDVEHLNVLRAIPDYIQDFRHGEKGETAMNSYFELYHYLMQRLMLKNTELDLSHWSGWIMRSGRPDRDLIQIAFVSLAYNLPRYRNLTKEHHFDDTVLQKIREKESLD

SEQ ID NO: 2 - DNA, 36 bp, synthetic construct
  source 1..36: mol_type = other DNA
ggaagataactctacaaacctgtagggttctgagac

SEQ ID NO: 3 - DNA, 36 bp, synthetic construct
  source 1..36: mol_type = other DNA
ggaagataactctacaaacctgtagagttctgagac

SEQ ID NO: 4 - DNA, 6793 bp, synthetic construct
  source 1..6793: mol_type = other DNA
cctgcaggcagctgcgcgctcgctcgctcactgaggccgcccgggcgtcgggcgacctttggtcgcccggcctcagtgagcgagcgagcgcgcagagagggagtggccaactccatcactaggggttcctgcggcctctagactcgaggcgttgacattgattattgactagttattaatagtaatcaattacggggtcattagttcatagcccatatatggagttccgcgttacataacttacggtaaatggcccgcctggctgaccgcccaacgacccccgcccattgacgtcaataatgacgtatgttcccatagtaacgccaatagggactttccattgacgtcaatgggtggagtatttacggtaaactgcccacttggcagtacatcaagtgtatcatatgccaagtacgccccctattgacgtcaatgacggtaaatggcccgcctggcattatgcccagtacatgaccttatgggactttcctacttggcagtacatctacgtattagtcatcgctattaccatggtgatgcggttttggcagtacatcaatgggcgtggatagcggtttgactcacggggatttccaagtctccaccccattgacgtcaatgggagtttgttttggcaccaaaatcaacgggactttccaaaatgtcgtaacaactccgccccattgacgcaaatgggcggtaggcgtgtacggtgggaggtctatataagcagagctctctggctaactaccggtgccaccatgccggcagctaagaaaaagaaactggatggcagcgtcgacatgagcaaggacaagaaaaccaaggccaagagaatgggcgtgaaggccctgctggcccacggcgaggacaagctgaccatgaccaccttcggcaagggcaacagaagcaagatcgagttcaccgagggctaccacggcagagccctggagacacccaagcacttcggcatcagaggcttcgaggtgagaagaatcgacgagaacgtggacctgtgcggcgacctggaggagggcaagaccatcgaggccctgctggtgaaccccagcgagaaggtgggcgaggactacctgaagctgaagggcaccctggagaagagattcttcggcagagagttcccccacgacaacatcagaatccagctgatctacaacatcctggacatctacaagatcctgggcatgaacgtggccgacatcctgtacgccctgggcaacatgcaggacaccgagctggacatcgacatgttcggccagagcctgaacaacgaggacaacctgaaggagtgcctgaagagaatgaggccctacatgggctacttcggcgacatcttcaagatcagccccaagggcgagaacatcgccgacagagagcacaacaagaaggtgctgagatgcatcagcgtgctgagaaacgccaccgcccacgacaagcaggacgagtacccctggttcaagagcagcgacatctacgagacaaagatcttcaaggccgacatgtggaagatcatcaaggaccagtacagagagaagatcaagaaggtgaacaaggacttcctgagcaagaacgccgtgaacatggccatcctgttcgacctgctgaacgccagagacgtggagcagaagaagcagatcaccgacgagttctacagattcaccatcagaaaggacggcaagaacctgggcatgaacctggtgaagatcagagagatcatcatcgacagatacgccagcggcctgagagacaagaagcacgacccccacagacagaagatcaacgtgatcgccgacttcctgatcttcagagccctgagccagaaccagggcatcatcgacaagaccgtgagcagcctgagactgaccaaggacgaggaggagaaggaccacgtgtaccagaacgccgccgagctggtgtggggcatggtgagcaactgcctgaccccctacttcaacgaccccaagaacaagtacatcctgaagtacaaggacgccaagacccccggcgacttcgaggactggatcaccagcaagatcagcgaggacgacggcgagcccttcgtgaaggtgctgagcttcctgtgcaacttcctggagggcaaggagatcaacgagctgctgaccgcctacatccacaagttcgagtgcatccaggacttcctgaacgtgatcagcagcctgggcgagaacgtgcagttccagcccagattcgccctgttcaacaacgccagcttcgcccagaacgtggccgtgcagctgagaatcctggccagcatcggcaagatgaagcccgacctgaccgaggccaagaggcccctgtacaaggccgccatcagaatgctgtgcccccccgagaagtgggagaagtacaccagcgacgagtggctggagaagaacatgctgctgaacagcgaggacagaaagaacgacaagaagaagaagcaggtgaaccccttcagaaacttcatcgccggcaacgtgatcgagagcagaagattcatgtacctggtgagatacagcaagcccaaggccgtgagagccatcatgcagaacagaagcatcgtgaactacgtgctgcacagactgcccagcgagcaggtgcacagatacgccagcgtgttccccgagaacttcgccgacctggagcaggagatcgacttcctgaccaagaagctgttcgagttcagcttcgaggagctgctgcacgagaaggacgtgatcctgaacaacagcagaagccacaagcccagcctggagatcgagagactgaaggccatcaccggcctgtacctgagcgtggcctacatcgccatcaagaacatcgtgaaggccaacgccagatactacatcgccttcgccgtgttcgagagagacaaggagctggtgaaggccaaggacgccagaatccagaccaagatccccgagacagacttccccgactacttctgcctgacccagtactacctggacagagacgaggagaagaagttccccggcgaccccagagacaaggaggccttcttcgagcacctgagaaagaccaagagacacttcagcaagcagtggagagagtggctgaacgagaagatcgccgacgccaagagcagccaggccaccggcctgctgctgagagaggccagaaacgacgtggagcacctgaacgtgctgagagccatccccgactacatccaggacttcagacacggcgagaagggcgagacagccatgaacagctacttcgagctgtaccactacctgatgcagagactgatgctgaagaacaccgagctggacctgagccactggagcggctggatcatgagaagcggcagacccgacagagacttgatccagatcgccttcgtgagcctggcctacaacctgcccagatacagaaacctgaccaaggagcaccacttcgacgacaccgtgctgcagaagatcagagagaaggagagcctggacacaggcggcggccccggcggcggcgccgccgccggcagcggcagccctaagaaaaaacgaaaagttggcagcggaagcaaaaggccggcggccacgaaaaaggccggccaggcaaaaaagaaaaagctcgagtacccatacgatgttccagattacgcttgagaattccccttgagcatctgacttctggctaataaaggaaatttattttcattgcaatagtgtgttggaattttttgtgtctctcaggtaccgagggcctatttcccatgattccttcatatttgcatatacgatacaaggctgttagagagataattggaattaatttgactgtaaacacaaagatattagtacaaaatacgtgacgtagaaagtaataatttcttgggtagtttgcagttttaaaattatgttttaaaatggactatcatatgcttaccgtaacttgaaagtatttcgatttcttggctttatatatcttgtggaaaggacgaaacaccggaagataactctacaaacctgtagggttctgagacggagaccacggcaggtctcattttttgcggccgcaggaacccctagtgatggagttggccactccctctctgcgcgctcgctcgctcactgaggccgggcgaccaaaggtcgcccgacgcccgggctttgcccgggcggcctcagtgagcgagcgagcgcgcagctgcctgcaggggcgcctgatgcggtattttctccttacgcatctgtgcggtatttcacaccgcatacgtcaaagcaaccatagtacgcgccctgtagcggcgcattaagcgcggcgggtgtggtggttacgcgcagcgtgaccgctacacttgccagcgccttagcgcccgctcctttcgctttcttcccttcctttctcgccacgttcgccggctttccccgtcaagctctaaatcgggggctccctttagggttccgatttagtgctttacggcacctcgaccccaaaaaacttgatttgggtgatggttcacgtagtgggccatcgccctgatagacggtttttcgccctttgacgttggagtccacgttctttaatagtggactcttgttccaaactggaacaacactcaactctatctcgggctattcttttgatttataagggattttgccgatttcggtctattggttaaaaaatgagctgatttaacaaaaatttaacgcgaattttaacaaaatattaacgtttacaattttatggtgcactctcagtacaatctgctctgatgccgcatagttaagccagccccgacacccgccaacacccgctgacgcgccctgacgggcttgtctgctcccggcatccgcttacagacaagctgtgaccgtctccgggagctgcatgtgtcagaggttttcaccgtcatcaccgaaacgcgcgagacgaaagggcctcgtgatacgcctatttttataggttaatgtcatgataataatggtttcttagacgtcaggtggcacttttcggggaaatgtgcgcggaacccctatttgtttatttttctaaatacattcaaatatgtatccgctcatgagacaataaccctgataaatgcttcaataatattgaaaaaggaagagtatgagtattcaacatttccgtgtcgcccttattcccttttttgcggcattttgccttcctgtttttgctcacccagaaacgctggtgaaagtaaaagatgctgaagatcagttgggtgcacgagtgggttacatcgaactggatctcaacagcggtaagatccttgagagttttcgccccgaagaacgttttccaatgatgagcacttttaaagttctgctatgtggcgcggtattatcccgtattgacgccgggcaagagcaactcggtcgccgcatacactattctcagaatgacttggttgagtactcaccagtcacagaaaagcatcttacggatggcatgacagtaagagaattatgcagtgctgccataaccatgagtgataacactgcggccaacttacttctgacaacgatcggaggaccgaaggagctaaccgcttttttgcacaacatgggggatcatgtaactcgccttgatcgttgggaaccggagctgaatgaagccataccaaacgacgagcgtgacaccacgatgcctgtagcaatggcaacaacgttgcgcaaactattaactggcgaactacttactctagcttcccggcaacaattaatagactggatggaggcggataaagttgcaggaccacttctgcgctcggcccttccggctggctggtttattgctgataaatctggagccggtgagcgtggaagccgcggtatcattgcagcactggggccagatggtaagccctcccgtatcgtagttatctacacgacggggagtcaggcaactatggatgaacgaaatagacagatcgctgagataggtgcctcactgattaagcattggtaactgtcagaccaagtttactcatatatactttagattgatttaaaacttcatttttaatttaaaaggatctaggtgaagatcctttttgataatctcatgaccaaaatcccttaacgtgagttttcgttccactgagcgtcagaccccgtagaaaagatcaaaggatcttcttgagatcctttttttctgcgcgtaatctgctgcttgcaaacaaaaaaaccaccgctaccagcggtggtttgtttgccggatcaagagctaccaactctttttccgaaggtaactggcttcagcagagcgcagataccaaatactgttcttctagtgtagccgtagttaggccaccacttcaagaactctgtagcaccgcctacatacctcgctctgctaatcctgttaccagtggctgctgccagtggcgataagtcgtgtcttaccgggttggactcaagacgatagttaccggataaggcgcagcggtcgggctgaacggggggttcgtgcacacagcccagcttggagcgaacgacctacaccgaactgagatacctacagcgtgagctatgagaaagcgccacgcttcccgaagggagaaaggcggacaggtatccggtaagcggcagggtcggaacaggagagcgcacgagggagcttccagggggaaacgcctggtatctttatagtcctgtcgggtttcgccacctctgacttgagcgtcgatttttgtgatgctcgtcaggggggcggagcctatggaaaaacgccagcaacgcggcctttttacggttcctggccttttgctggccttttgctcacatgt

SEQ ID NO: 5 - DNA, 25 bp, synthetic construct
  source 1..25: mol_type = other DNA
cagccgcagccgtccagcacgaggc

SEQ ID NO: 6 - DNA, 25 bp, synthetic construct
  source 1..25: mol_type = other DNA
gcgaggaggaccacgaaggcgacgc

SEQ ID NO: 7 - DNA, 25 bp, synthetic construct
  source 1..25: mol_type = other DNA
tcgcgctcggtgcacagctcgccca

SEQ ID NO: 8 - DNA, 25 bp, synthetic construct
  source 1..25: mol_type = other DNA
cgtcacacacccactcctcgcagca

SEQ ID NO: 9 - DNA, 25 bp, synthetic construct
  source 1..25: mol_type = other DNA
aatcatagttgggtctgggccaaac

SEQ ID NO: 10 - DNA, 25 bp, synthetic construct
  source 1..25: mol_type = other DNA
agacgaacgtccatgctgcacaggg

SEQ ID NO: 11 - DNA, 25 bp, synthetic construct
  source 1..25: mol_type = other DNA
tctcttccaggtcagcttcgcaagg

SEQ ID NO: 12 - DNA, 25 bp, synthetic construct
  source 1..25: mol_type = other DNA
accgaagatgcagggagcaccatct

SEQ ID NO: 13 - DNA, 25 bp, synthetic construct
  source 1..25: mol_type = other DNA
ttcaaagatgtcattgtctccggga

SEQ ID NO: 14 - RNA, 2338 nt, Homo sapiens
  source 1..2338: mol_type = other RNA
acacaacaactcttccccgctgagaggagacagccagtgcgactccaccctccagctcgacggcagccgccccggccgacagccccgagacgacagcccggcgcgtcccggtccccacctccgaccaccgccagcgctccaggccccgccgctccccgctcgccgccaccgcgccctccgctccgcccgcagtgccaaccatgaccgccgccagtatgggccccgtccgcgtcgccttcgtggtcctcctcgccctctgcagccggccggccgtcggccagaactgcagcgggccgtgccggtgcccggacgagccggcgccgcgctgcccggcgggcgtgagcctcgtgctggacggctgcggctgctgccgcgtctgcgccaagcagctgggcgagctgtgcaccgagcgcgacccatgcgacccgcacaagggcctattctgtcacttcggctccccggccaaccgcaagatcggcgtgtgcaccgccaaagatggtgctccctgcatcttcggtggtacggtgtaccgcagcggagagtccttccagagcagctgcaagtaccagtgcacgtgcctggacggggcggtgggctgcatgcccctgtgcagcatggacgttcgtctgcccagccctgactgccccttcccgaggagggtcaagctgcccgggaaatgctgcgaggagtgggtgtgtgacgagcccaaggaccaaaccgtggttgggcctgccctcgcggcttaccgactggaagacacgtttggcccagacccaactatgattagagccaactgcctggtccagaccacagagtggagcgcctgttccaagacctgtgggatgggcatctccacccgggttaccaatgacaacgcctcctgcaggctagagaagcagagccgcctgtgcatggtcaggccttgcgaagctgacctggaagagaacattaagaagggcaaaaagtgcatccgtactcccaaaatctccaagcctatcaagtttgagctttctggctgcaccagcatgaagacataccgagctaaattctgtggagtatgtaccgacggccgatgctgcaccccccacagaaccaccaccctgccggtggagttcaagtgccctgacggcgaggtcatgaagaagaacatgatgttcatcaagacctgtgcctgccattacaactgtcccggagacaatgacatctttgaatcgctgtactacaggaagatgtacggagacatggcatgaagccagagagtgagagacattaactcattagactggaacttgaactgattcacatctcatttttccgtaaaaatgatttcagtagcacaagttatttaaatctgtttttctaactgggggaaaagattcccacccaattcaaaacattgtgccatgtcaaacaaatagtctatcaaccccagacactggtttgaagaatgttaagacttgacagtggaactacattagtacacagcaccagaatgtatattaaggtgtggctttaggagcagtgggagggtaccagcagaaaggttagtatcatcagatagcatcttatacgagtaatatgcctgctatttgaagtgtaattgagaaggaaaattttagcgtgctcactgacctgcctgtagccccagtgacagctaggatgtgcattctccagccatcaagagactgagtcaagttgttccttaagtcagaacagcagactcagctctgacattctgattcgaatgacactgttcaggaatcggaatcctgtcgattagactggacagcttgtggcaagtgaatttgcctgtaacaagccagattttttaaaatttatattgtaaatattgtgtgtgtgtgtgtgtgtgtatatatatatatatgtacagttatctaagttaatttaaagttgtttgtgcctttttatttttgtttttaatgctttgatatttcaatgttagcctcaatttctgaacaccataggtagaatgtaaagcttgtctgatcgttcaaagcatgaaatggatacttatatggaaattctgctcagatagaatgacagtccgtcaaaacagattgtttgcaaaggggaggcatcagtgtccttggcaggctgatttctaggtaggaaatgtggtagcctcacttttaatgaacaaatggcctttattaaaaactgagtgactctatatagctgatcagttttttcacctggaagcatttgtttctactttgatatgactgtttttcggacagtttatttgttgagagtgtgaccaaaagttacatgtttgcacctttctagttgaaaataaagtgtatattttttctataaa

SEQ ID NO: 15 - DNA, 9582 bp, synthetic construct
  source 1..9582: mol_type = other DNA
gtcgacggatcgggagatctcccgatcccctatggtgcactctcagtacaatctgctctgatgccgcatagttaagccagtatctgctccctgcttgtgtgttggaggtcgctgagtagtgcgcgagcaaaatttaagctacaacaaggcaaggcttgaccgacaattgcatgaagaatctgcttagggttaggcgttttgcgctgcttcgcgatgtacgggccagatatacgcgttgacattgattattgactagttattaatagtaatcaattacggggtcattagttcatagcccatatatggagttccgcgttacataacttacggtaaatggcccgcctggctgaccgcccaacgacccccgcccattgacgtcaataatgacgtatgttcccatagtaacgccaatagggactttccattgacgtcaatgggtggagtatttacggtaaactgcccacttggcagtacatcaagtgtatcatatgccaagtacgccccctattgacgtcaatgacggtaaatggcccgcctggcattatgcccagtacatgaccttatgggactttcctacttggcagtacatctacgtattagtcatcgctattaccatggtgatgcggttttggcagtacatcaatgggcgtggatagcggtttgactcacggggatttccaagtctccaccccattgacgtcaatgggagtttgttttggcaccaaaatcaacgggactttccaaaatgtcgtaacaactccgccccattgacgcaaatgggcggtaggcgtgtacggtgggaggtctatagaccagatctgagcctgggagctctctggctaactagggaacccactgcttaagcctcaataaagcttgccttgagtgcttcaagtagtgtgtgcccgtctgttgtgtgactctggtaactagagatccctcagacccttttagtcagtgtggaaaatctctagcagtggcgcccgaacagggacttgaaagcgaaagggaaaccagaggagctctctcgacgcaggactcggcttgctgaagcgcgcacggcaagaggcgaggggcggcgactggtgagtacgccaaaaattttgactagcggaggctagaaggagagagatgggtgcgagagcgtcagtattaagcgggggagaattagatcgcgatgggaaaaaattcggttaaggccagggggaaagaaaaaatataaataaacatatagtatgggcaagcagggagctagaacgattcgcagttaatcctggcctgttagaaacatcagaaggctgtagacaaatactgggacagctacaaccatcccttcagacaggatcagaagaacttagatcattatataatacagtagcaaccctctattgtgtgcatcaaaggatagagataaaagacaccaaggaagctttagacaagatagaggaagagcaaaacaaaagtaagaccaccgcacagcaagcggccggccgcgctgatcttcagacctggaggaggagatatgagggacaattggagaagtgaattatataaatataaagtagtaaaaattgaaccattaggagtagcacccaccaaggcaaagagaagagtggtgcagagagaaaaaagagcagtgggaataggagctttgttccttgggttcttgggagcagcaggaagcactatgggcgcagcgtcaatgacgctgacggtacaggccagacaattattgtctggtatagtgcagcagcagaacaatttgctgagggctattgaggcgcaacagcatctgttgcaactcacagtctggggcatcaagcagctccaggcaagaatcctggctgtggaaagatacctaaaggatcaacagctcctggggatttggggttgctctggaaaactcatttgcaccactgctgtgccttggaatgctagttggagtaataaatctctggaacagatttggaatcacacgacctggatggagtgggacagagaaattaacaattacacaagcttaatacactccttaattgaagaatcgcaaaaccagcaagaaaagaatgaacaagaattattggaattagataaatgggcaagtttgtggaattggtttaacataacaaattggctgtggtatataaaattattcataatgatagtaggaggcttggtaggtttaagaatagtttttgctgtactttctatagtgaatagagttaggcagggatattcaccattatcgtttcagacccacctcccaaccccgaggggacccgacaggcccgaaggaatagaagaagaaggtggagagagagacagagacagatccattcgattagtgaacggatcggcactgcgtgcgccaattctgcagacaaatggcagtattcatccacaattttaaaagaaaaggggggattggggggtacagtgcaggggaaagaatagtagacataatagcaacagacatacaaactaaagaattacaaaaacaaattacaaaaattcaaaattttcgggtttattacagggacagcagagatccagtttggttagtaccgggcccgctctagcgtcgaggagcttggcccattgcatacgttgtatccatatcataatatgtacatttatattggctcatgtccaacattaccgccatgttgacattgattattgactagttattaatagtaatcaattacggggtcattagttcatagcccatatatggagttccgcgttacataacttacggtaaatggcccgcctggctgaccgcccaacgacccccgcccattgacgtcaataatgacgtatgttcccatagtaacgccaatagggactttccattgacgtcaatgggtggagtatttacggtaaactgcccacttggcagtacatcaagtgtatcatatgccaagtacgccccctattgacgtcaatgacggtaaatggcccgcctggcattatgcccagtacatgaccttatgggactttcctacttggcagtacatctacgtattagtcatcgctattaccatggtgatgcggttttggcagtacatcaatgggcgtggatagcggtttgactcacggggatttccaagtctccaccccattgacgtcaatgggagtttgttttggcaccaaaatcaacgggactttccaaaatgtcgtaacaactccgccccattgacgcaaatgggcggtaggcgtgtacggtgggaggtctatataagcagagctcgtttagtgaaccgtcagatcgcctggagacgccatccacgctgttttgacctccatagaagacaccgggaccgatccagcctccgcggccccgaattcgccaccatggccatgaccgccgccagtatgggccccgtccgcgtcgccttcgtggtcctcctcgccctctgcagccggccggccgtcggccagaactgcagcgggccgtgccggtgcccggacgagccggcgccgcgctgcccggcgggcgtgagcctcgtgctggacggctgcggctgctgccgcgtctgcgccaagcagctgggcgagctgtgcaccgagcgcgacccatgcgacccgcacaagggcctattctgtcacttcggctccccggccaaccgcaagatcggcgtgtgcaccgccaaagatggtgctccctgcatcttcggtggtacggtgtaccgcagcggagagtccttccagagcagctgcaagtaccagtgcacgtgcctggacggggcggtgggctgcatgcccctgtgcagcatggacgttcgtctgcccagccctgactgccccttcccgaggagggtcaagctgcccgggaaatgctgcgaggagtgggtgtgtgacgagcccaaggaccaaaccgtggttgggcctgccctcgcggcttaccgactggaagacacgtttggcccagacccaactatgattagagccaactgcctggtccagaccacagagtggagcgcctgttccaagacctgtgggatgggcatctccacccgggttaccaatgacaacgcctcctgcaggctagagaagcagagccgcctgtgcatggtcaggccttgcgaagctgacctggaagagaacattaagaagggcaaaaagtgcatccgtactcccaaaatctccaagcctatcaagtttgagctttctggctgcaccagcatgaagacataccgagctaaattctgtggagtatgtaccgacggccgatgctgcaccccccacagaaccaccaccctgccggtggagttcaagtgccctgacggcgaggtcatgaagaagaacatgatgttcatcaagacctgtgcctgccattacaactgtcccggagacaatgacatctttgaatcgctgtactacaggaagatgtacggagacatggcaggatccgctagcggcagtggagagggcagaggaagtctgctaacatgcggtgacgtcgaggagaatcctggcccagtgagcaagggcgaggagctgttcaccggggtggtgcccatcctggtcgagctggacggcgacgtaaacggccacaagttcagcgtgtccggcgagggcgagggcgatgccacctacggcaagctgaccctgaagttcatctgcaccaccggcaagctgcccgtgccctggcccaccctcgtgaccaccctgacctacggcgtgcagtgcttcagccgctaccccgaccacatgaagcagcacgacttcttcaagtccgccatgcccgaaggctacgtccaggagcgcaccatcttcttcaaggacgacggcaactacaagacccgcgccgaggtgaagttcgagggcgacaccctggtgaaccgcatcgagctgaagggcatcgacttcaaggaggacggcaacatcctggggcacaagctggagtacaactacaacagccacaacgtctatatcatggccgacaagcagaagaacggcatcaaggtgaacttcaagatccgccacaacatcgaggacggcagcgtgcagctcgccgaccactaccagcagaacacccccatcggcgacggccccgtgctgctgcccgacaaccactacctgagcacccagtccgccctgagcaaagaccccaacgagaagcgcgatcacatggtcctgctggagttcgtgaccgccgccgggatcactctcggcatggacgagctgtacaagtaaggatcctaggcggccgcgcatgccctgcaggtgatctatcgatcggccggcccctctccctccccccccccctaacgttactggccgaagccgcttggaataaggccggtgtgcgtttgtctatatgttattttccaccatattgccgtcttttggcaatgtgagggcccggaaacctggccctgtcttcttgacgagcattcctaggggtctttcccctctcgccaaaggaatgcaaggtctgttgaatgtcgtgaaggaagcagttcctctggaagcttcttgaagacaaacaacgtctgtagcgaccctttgcaggcagcggaaccccccacctggcgacaggtgcctctgcggccaaaagccacgtgtataagatacacctgcaaaggcggcacaaccccagtgccacgttgtgagttggatagttgtggaaagagtcaaatggctctcctcaagcgtattcaacaaggggctgaaggatgcccagaaggtaccccattgtatgggatctgatctggggcctcggtacacatgctttacatgtgtttagtcgaggttaaaaaaacgtctaggccccccgaaccacggggacgtggttttcctttgaaaaacacgatgataatatggccacaaccgggccggatatcacgcgtgatctgatcagcacgtgttgacaattaatcatcggcatagtatatcggcatagtataatacgacaaggtgaggaactaaaccatggccaagcctttgtctcaagaagaatccaccctcattgaaagagcaacggctacaatcaacagcatccccatctctgaagactacagcgtcgccagcgcagctctctctagcgacggccgcatcttcactggtgtcaatgtatatcattttactgggggaccttgtgcagaactcgtggtgctgggcactgctgctgctgcggcagctggcaacctgacttgtatcgtcgcgatcggaaatgagaacaggggcatcttgagcccctgcggacggtgccgacaggtgcttctcgatctgcatcctgggatcaaagccatagtgaaggacagtgatggacagccgacggcagttgggattcgtgaattgctgccctctggttatgtgtgggagggctaagcaatgcatacatgtgtttaaacctcgacttaattaagtcgagggtcgacggtatcgataagctcgcttcacgagatcatgtttaagggttccggttccactaggtacaattcgatatcaagcttatcgataatcaacctctggattacaaaatttgtgaaagattgactggtattcttaactatgttgctccttttacgctatgtggatacgctgctttaatgcctttgtatcatgctattgcttcccgtatggctttcattttctcctccttgtataaatcctggttgctgtctctttatgaggagttgtggcccgttgtcaggcaacgtggcgtggtgtgcactgtgtttgctgacgcaacccccactggttggggcattgccaccacctgtcagctcctttccgggactttcgctttccccctccctattgccacggcggaactcatcgccgcctgccttgcccgctgctggacaggggctcggctgttgggcactgacaattccgtggtgttgtcggggaaatcatcgtcctttccttggctgctcgcctgtgttgccacctggattctgcgcgggacgtccttctgctacgtcccttcggccctcaatccagcggaccttccttcccgcggcctgctgccggctctgcggcctcttccgcgtcttcgccttcgccctcagacgagtcggatctccctttgggccgcctccccgcatcgataccgtcgacctcgatcgagacctagaaaaacatggagcaatcacaagtagcaatacagcagctaccaatgctgattgtgcctggctagaagcacaagaggaggaggaggtgggttttccagtcacacctcaggtacctttaagaccaatgacttacaaggcagctgtagatcttagccactttttaaaagaaaaggggggactggaagggctaattcactcccaacgaagacaagatatccttgatctgtggatctaccacacacaaggctacttccctgattggcagaactacacaccagggccagggatcagatatccactgacctttggatggtgctacaagctagtaccagttgagcaagagaaggtagaagaagccaatgaaggagagaacacccgcttgttacaccctgtgagcctgcatgggatggatgacccggagagagaagtattagagtggaggtttgacagccgcctagcatttcatcacatggcccgagagctgcatccggactgtactgggtctctctggttagaccagatctgagcctgggagctctctggctaactagggaacccactgcttaagcctcaataaagcttgccttgagtgcttcaagtagtgtgtgcccgtctgttgtgtgactctggtaactagagatccctcagacccttttagtcagtgtggaaaatctctagcagcatgtgagcaaaaggccagcaaaaggccaggaaccgtaaaaaggccgcgttgctggcgtttttccataggctccgcccccctgacgagcatcacaaaaatcgacgctcaagtcagaggtggcgaaacccgacaggactataaagataccaggcgtttccccctggaagctccctcgtgcgctctcctgttccgaccctgccgcttaccggatacctgtccgcctttctcccttcgggaagcgtggcgctttctcatagctcacgctgtaggtatctcagttcggtgtaggtcgttcgctccaagctgggctgtgtgcacgaaccccccgttcagcccgaccgctgcgccttatccggtaactatcgtcttgagtccaacccggtaagacacgacttatcgccactggcagcagccactggtaacaggattagcagagcgaggtatgtaggcggtgctacagagttcttgaagtggtggcctaactacggctacactagaagaacagtatttggtatctgcgctctgctgaagccagttaccttcggaaaaagagttggtagctcttgatccggcaaacaaaccaccgctggtagcggtggtttttttgtttgcaagcagcagattacgcgcagaaaaaaaggatctcaagaagatcctttgatcttttctacggggtctgacgctcagtggaacgaaaactcacgttaagggattttggtcatgagattatcaaaaaggatcttcacctagatccttttaaattaaaaatgaagttttaaatcaatctaaagtatatatgagtaaacttggtctgacagttaccaatgcttaatcagtgaggcacctatctcagcgatctgtctatttcgttcatccatagttgcctgactccccgtcgtgtagataactacgatacgggagggcttaccatctggccccagtgctgcaatgataccgcgagacccacgctcaccggctccagatttatcagcaataaaccagccagccggaagggccgagcgcagaagtggtcctgcaactttatccgcctccatccagtctattaattgttgccgggaagctagagtaagtagttcgccagttaatagtttgcgcaacgttgttgccattgctacaggcatcgtggtgtcacgctcgtcgtttggtatggcttcattcagctccggttcccaacgatcaaggcgagttacatgatcccccatgttgtgcaaaaaagcggttagctccttcggtcctccgatcgttgtcagaagtaagttggccgcagtgttatcactcatggttatggcagcactgcataattctcttactgtcatgccatccgtaagatgcttttctgtgactggtgagtactcaaccaagtcattctgagaatagtgtatgcggcgaccgagttgctcttgcccggcgtcaatacgggataataccgcgccacatagcagaactttaaaagtgctcatcattggaaaacgttcttcggggcgaaaactctcaaggatcttaccgctgttgagatccagttcgatgtaacccactcgtgcacccaactgatcttcagcatcttttactttcaccagcgtttctgggtgagcaaaaacaggaaggcaaaatgccgcaaaaaagggaataagggcgacacggaaatgttgaatactcatactcttcctttttcaatattattgaagcatttatcagggttattgtctcatgagcggatacatatttgaatgtatttagaaaaataaacaaataggggttccgcgcacatttccccgaaaagtgccacctgac

SEQ ID NO: 16 - DNA, 20 bp, synthetic construct
  source 1..20: mol_type = other DNA
gcgtgtgcaccgccaaagat

SEQ ID NO: 17 - DNA, 20 bp, synthetic construct
  source 1..20: mol_type = other DNA
aacgtccatgctgcacaggg

SEQ ID NO: 18 - DNA, 19 bp, synthetic construct
  source 1..19: mol_type = other DNA
cagcatggacgttcgtctg

SEQ ID NO: 19 - DNA, 20 bp, synthetic construct
  source 1..20: mol_type = other DNA
aaccacggtttggtccttgg

SEQ ID NO: 20 - DNA, 20 bp, synthetic construct
  source 1..20: mol_type = other DNA
ccatggggaaggtgaaggtc

SEQ ID NO: 21 - DNA, 21 bp, synthetic construct
  source 1..21: mol_type = other DNA
gaaggggtcattgatggcaac

SEQ ID NO: 22 - RNA, 4910 nt, Homo sapiens
  source 1..4910: mol_type = other RNA
gcgagccggcgagcgggcagagctcggcactgcgccggggcgcacggctcgggggacccaggcccagctaccttccctccgcccccgggctctgttctcactttccagcagtggaaggacgggaagcgggagccatgcagtccgaatcggggatcgtgccggatttcgaagtcggggaggagtttcatgaagagcccaaaacctattacgaactcaaaagtcaaccgctgaagagcagaaagtcagatggctttgtgttgtttgacgtggttccttttccaaatagatgactgtaaagatgacctgatgatcctatggactgggctataaactttgtgcatctcccttcttgtgccttaatggcaagcagttccgccgagcatcctggggcctccaagcctccgataagctcctccagtatgacatcacgcatcttgctacgccagcaactcatgcgtgagcagatgcaggagcaggagcgcagggagcagcagcagaagctgcaggcggcccagttcatgcaacagagagtgcccgtgagtcagacaccagccataaacgtcagtgtgcccaccacccttccctctgccacgcaggtgccgatggaagtccttaaggtgcagacccacctcgaaaaccccaccaagtaccacatacagcaagcccaacggcagcaggtaaagcagtacctttctaccactttagcaaataaacatgccaaccaagtcctgagcttgccatgtccaaaccagcctggcgatcatgtcatgccaccggtgccggggagcagcgcacccaacagccccatggctatgcttacgcttaactccaactgtgaaaaagagggattttataagtttgaagagcaaaacagggcagagagcgagtgcccaggcatgaacacacattcacgagcgtcctgtatgcagatggatgatgtaatcgatgacatcattagcctagaatcaagttataatgaggaaatcttgggcttgatggatcctgctttgcaaatggcaaatacgttgcctgtctcgggaaacttgattgatctttatggaaaccaaggtctgcccccaccaggcctcaccatcagcaactcctgtccagccaaccttcccaacataaaaagggagctcacagagtctgaagcaagagcactggccaaagagaggcagaaaaaggacaatcacaacctgattgaacgaagaagaagatttaacataaatgaccgcattaaagaactaggtactttgattcccaagtcaaatgatccagacatgcgctggaacaagggaaccatcttaaaagcatccgtggactatatccgaaagttgcaacgagaacagcaacgcgcaaaagaacttgaaaaccgacagaagaaactggagcacgccaaccggcatttgttgctcagaatacaggaacttgaaatgcaggctcgagctcatggactttcccttattccatccacgggtctctgctctccagatttggtgaatcggatcatcaagcaagaacccgttcttgagaactgcagccaagacctccttcagcatcatgcagacctaacctgtacaacaactctcgatctcacggatggcaccatcaccttcaacaacaacctcggaactgggactgaggccaaccaagcctatagtgtccccacaaaaatgggatccaaactggaagacatcctgatggacgacaccctttctcccgtcggtgtcactgatccactcctttcctcagtgtcccccggagcttccaaaacaagcagccggaggagcagtatgagcatggaagagacggagcacacttgttagcgaatcctccctgcactgcattcgcacaaactgcttcctttcttgattcgtagatttaataacttacctgaaggggttttcttgataattttcctttaatatgaaattttttttcatgctttatcaatagcccaggatatattttatttttagaattttgtgaaacagacttgtatattctattttacaactacaaatgcctccaaagtattgtacaaataagtgtgcagtatctgtgaactgaattcaccacagactttagctttctgagcaagaggattttgcgtcagagaaatgtctgtccatttttattcaggggaaacttgatttgagatttttatgcctgtgacttccttggaaatcaaatgtaaagtttaattgaaagaatgtaaagcaaccaaaaagaaaaaaaaaaagaaagaaagaggaaaagaaatccatactaacccttttccattttataaatgtattgattcattggtactgccttaaagatacagtacccctctagctttgtttagtctttatactgcaaactatttaaagaaatatgtattctgtaaaagaaaaaaaaaatgcggccttttcatgaggatcgtctggttagaaaacataactgataccaaccgaaactgaagggagttagaccaaggctctgaaatataaagtctaatcttgctctcttttattctgtgctgttacagttttcttcatcaatgagtgtgatccagtttttcataagatattttattttgaaatggaaattaatgtcctctcaaagtaaaatattgaggagcactgaaagtatgttttactttttttttattttatttttgcttttgataagaaaaccgaactgggcatatttctaattggctttactatttttatttttaaattatgttttactgttcatttgatttgtacagattctttattatcattgttcttttcaatatatttgtattaatttgtaagaatatgcatcttaaaatggcaagttttccatatttttacaactcactggtggttttccgcattctttgtacacccatgaaagaaaacttttatgcaaggtcttgcatttaaaagacagctttgcgaatattttgtaaattacagtctcactcagaactgtttttggacacatttaaggtgtagtattaataggttaaaaccaggctttctagaaagaataaacttacatatttatttttaggacatgaaaatagcaatattcttggagattgataaccatagcattaatacgcccattatggtcatttaaattggggtttatttcagcaaacttgttgaatttatttttaagaaagaaatactgtattgggaagttactgttacttgataacaatgttttaacaagaagcaatgttataaagttagtttcagtgcattatctacttgtgtagtcctatgcaataacagtagtgttacatgtatcaagcctagatgttttatacagatgccatatagtgttatgagccaggctgttgaatggaatttctcagtagcagcctacaactgaatagcaagtggcataaagcatatccattcagaatgaagtgccttaaatatagcagtagtcttttttggactagcactgactgaactgtaatgtaggggaaagtttcatgatggtatctatagtcaagacgaacatgtagcatggtgcctatgtagacaatataagagcttccaattttccttcagatatttttaatattaaatatattttagtgacagagtgccaacttctttcatcaggaaaccttattcaggagggtttttaaaaagtgtttaaatgtcaaatgtgaattggtgatgggtgatggagggttcagagaggagtgatcgtcagatgtgtgaatggacggtttaggtgaaaataatcaactgcatagttcccatgcacgctgggcaatgagaatccttggaaacattggtgatgctatcagttttatagctttatttcttaagggggtagggaaaattagttcccattctttcaacccccttaactgtatagctcttttcctagaatagtgacgcaaatctgcatgaacagctaattgtaccatagtgttcattgatacaatcatagcattgtctatttttctcttcatatttatatgggggggagggcgctggatgcaaaagttgaagatcgtgatgctatgatgttagttttccttagctgattttgagggtttttaaaaataaagcaaggttgactaacctacggccacgggaacaggaccatggttaagcaaccatatagaaagctttgttgaaagaaagtatggcatcttgtaccactgccctgactgtcacaactcctaaccttgccattgcctgcctccccctccccttctccttaagagacaatttctgcaggtggcaggtgagcaagcccaggagaatgctgcaatcttgggggtggttttatttatttcttttttgccaaatagagtgtggattcatttcaggggctagctaagccaagaggcagtggtttgggcttgttgtttgtaacaagaaaatgatccacaccactcccccgattcccgggtgcagaattgtaactcggggttgggcctctatatggagtgaccaaaatgccaaaattgtccatctgcctctgagtagggcaatggaaataccaaaccttctgactttgccaaaaagcatacaagcaacctggtcatacataggatgacaaaattctttctggttgtttttaaacaataaagcaataagaacaaatacaatacataggaagttaaaagcacaaaggaatgaacttattaatatttttgaaaaatgcactgggaaaaagttgatgtcaataacagtataaaacagccctatttcttgataaaaaatgacaaatgactgtctcttgcggatgcttggtactgtaatgttaataatagtcacctgctgttggatgcagcaataatttctgtatggtccatagcactgtatattatggatcgatattaatgtatccaatgaaataatcgacttgttcttgatagcctcattaaagcatttggtttttca

SEQ ID NO: 23 - RNA, 25 nt, synthetic construct
  source 1..25: mol_type = other RNA
cctgctcctgcatctgctcacgcat

SEQ ID NO: 24 - RNA, 25 nt, synthetic construct
  source 1..25: mol_type = other RNA
gcacactgacgtttatggctggtgt

SEQ ID NO: 25 - RNA, 25 nt, synthetic construct
  source 1..25: mol_type = other RNA
tgatgtcatactggaggagcttatc

SEQ ID NO: 26 - RNA, 25 nt, synthetic construct
  source 1..25: mol_type = other RNA
cactctctgttgcatgaactgggcc

SEQ ID NO: 27 - RNA, 25 nt, synthetic construct
  source 1..25: mol_type = other RNA
ccatcggcacctgcgtggcagaggg

SEQ ID NO: 28 - RNA, 25 nt, synthetic construct
  source 1..25: mol_type = other RNA
cagcttctgctgctgctccctgcgc

SEQ ID NO: 29 - RNA, 25 nt, synthetic construct
  source 1..25: mol_type = other RNA
tgagttgctggcgtagcaagatgcg

SEQ ID NO: 30 - RNA, 25 nt, synthetic construct
  source 1..25: mol_type = other RNA
aggccccaggatgctcggcggaact

SEQ ID NO: 31 - RNA, 25 nt, synthetic construct
  source 1..25: mol_type = other RNA
ccataggatcatcaggtcatcttta

SEQ ID NO: 32 - RNA, 25 nt, synthetic construct
  source 1..25: mol_type = other RNA
cttgccattaaggcacaagaaggga

SEQ ID NO: 33 - DNA, 20 bp, synthetic construct
  source 1..20: mol_type = other DNA
gcctccaagcctccgataag

SEQ ID NO: 34 - DNA, 21 bp, synthetic construct
  source 1..21: mol_type = other DNA
gcactctctgttgcatgaact

SEQ ID NO: 35 - RNA, 4654 nt, Homo sapiens
  source 1..4654: mol_type = other RNA
tgaaacaacctagtgagatccagtacagcttccaacttatattagaccaactttcctccctatgacattaatagctggggtatggagctgtcagagtgacacgtaaactccaatcagatcaccaagtggcctcagaaatgcacacatacaagctaaagaaaatagtcattctcttcttaaagtattaagatccaggccaaaggaaatggaatagctagcggctgtttaaaatgtgggaaacatagcactgctaaccagttatccactccaaatgagaaatgtgatgtgctagaaaacatattggagaaacatggttgggttctagaggaatgcagtgtctaaagctctagcagccttgggtagccttgggagttgggagtgggaaccatgcttaggaagcaactggagaaaagaagcctaatgcaaccatgagatcctggagcctgacatacaggacatttgtgtactcactgctcaatcgagggaggccttatccagctatactcattctcagaggcactgccttctgcactggaaatggagtccttcaaggctactatctgatttactgtgctgaataccctgatgggtggtacacagacatacggtttagcttgggtgtcttcttatttattttgggaatgggaataaacattcatagtgactatatattgcgccagctcaggaagcctggagaaatcagctacaggattccacaaggtggcttgtttacgtatgtttctggagccaatttcctcggtgagatcattgaatggatcggctatgccctggccacttggtccctcccagcacttgcatttgcatttttctcactttgtttccttgggctgcgagcttttcaccaccataggttctacctcaagatgtttgaggactaccccaaatctcggaaagcccttattccattcatcttttaaaggaaccaaattaaaaaggagcagagctcccacaatgctgatgaaaactgtcaagctgctgaaactgtaattttcatgatataatagtcccgtatatatgtaatagtaggtctcctggcgttctgccagctggcctggggattctgagtggtgtctgcttagagtttactcctacccttccagggacccctatcctgatccccaactgaagcttcaaaaagccacttttccaaatggcgacagttgcttcttagctattgctctgagaaagtacaaacttctcctatgtctttcaccgggcaatccaagtacatgtggcttcatacccactccctgtcaatgcaggacaactctgtaatcaagaattttttgacttgaaggcagtacttatagaccttattaaaggtatgcattttatacatgtaacagagtagcagaaatttaaactctgaagccacaaagacccagagcaaacccactcccaaatgaaaaccccagtcatggcttcctttttcttggttaattaggaaagatgagaaattattaggtagaccttgaatacaggagccctctcctcatagtgctgaaaagatactgatgcattgacctcatttcaaatttgtgcagtgtcttagttgatgagtgcctctgttttccagaagatttcacaatccccggaaaactggtatggctattcttgaaggccaggttttaataaccacaaacaaaaaggcatgaacctgggtggcttatgagagagtagagaacaacatgaccctggatggctactaagaggatagagaacagttttacaatagacattgcaaactctcatgtttttggaaactagtggcaatatccaaataatgagtagtgtaaaacaaagagaattaatgatgaggttacatgctgcttgcctccaccagatgtccacaacaatatgaagtacagcagaagccccaagcaactttcctttcctggagcttcttccttgtagttctcaggacctgttcaagaaggtgtctcctaggggcagcctgaatgcctccctcaaaggacctgcaggcagagactgaaaattgcagacagaggggcacgtctgggcagaaaacctgttttgtttggctcagacatatagttttttttttttttacaaagtttcaaaaacttaaaaatcaggagattccttcataaaactctagcattctagtttcatttaaaaagttggaggatctgaacatacagagcccacatttccacaccagaactggaactacgtagctagtaagcatttgagtttgcaaactcttgtgaaggggtcaccccagcatgagtgctgagatatggactctctaaggaaggggccgaacgcttgtaattggaatacatggaaatatttgtcttctcaggcctatgtttgcggaatgcattgtcaatatttagcaaactgttttgacaaatgagcaccagtggtactaagcacagaaactcactatataagtcacataggaaacttgaaaggtctgaggatgatgtagattactgaaaaatgcaaattgcaatcatataaataagtgtttttgttgttcattaaatacctttaaatcatggatgttaagcagttttgtttgaattaaaatatcctgggacttctggagattttcacaaggtattggggtgtgcttccctgtcccgcctgtccctcattcccattcaccctgtctgtagtgtcgtttcctttcttctcttctctcttcatgaaattaggggctgtgtgctggaaataaagaagtatgacttatacagcctctcagccacaattcagaactacaaggaagtacaataaaggtgcaggaaaacgtcatgaggttagatgccactcctggtgctgaggaatacacagggggaatgaacacacttggtgaagtaaatcttcaggtgtagcttgagctctgtgacataaaagacttccagttctctccatgacattgaaaactaccttgcttaagtcctttattttactaccatgtaaaacatccaggccggtccttgagatgaaataaatatacaataaatggcagtactcagtctcaggacaaaaccgccatttggcaatttcactttttgccacaagagggcgctttctaaaatagtatttagtccaaccttgacttaattaggtccaaccccagtcctgttgcctgatcgtggacctttcaagttagcatgatcgtggaacttcttaatctgaatatagggtagagtagcgtgaactctatgaaagctgaaaccttcccttgataattcaggtattctcagtgttctagggctgttgtgttcaatgacagtttgtcattgtttagggctaggatatgtatgtggattaaatacagtaaaggtctgaacatgtgctcatctctaaacatatttcttcccacttttaaaaatagggtgcaacaaaattatagttaattgaggtttccatggactgttttttggctaaaataatctaacagtgtcctagctcacaagatactctatcttggtcttgctgaagctttcacggaagaggcgttttcctgccaaccttgaagaaaatgttgagttttgtttgtttttcagaatttagacttaaagagctgaagcagacctcagacatcagctattcctaccacttcacattataggtagtgacactgagacccacagagttaaaaggcctcctcacagctggtacagagctggtcagagcagccatctcattttgtccctttgagggtcagatgtatgcttcttctgcttaaggcacagcctttagggctgccatctggatttctacagagctcatgcaggagaaaaatagccagagcttaagtgctgttgcatagttcagtttatacacctattgtcccatgcctgtttgtgtgtgaggcttccctcgctccgtgggagcaccaggctcatgccctttcataaacctatttgacagaatagagagttttccctcattggtgtagtcaagacaacatgtgtgttcagcatggaaaaaaggtttcaggtcataaacccccttatccctaatgcttactttcataaagaacaacagtggctccactgtattctaaaaggaaaaaggagctctaatgagaaatacgcaattaaacagctatttaggcggcttagaccctttcaggaacaaataaataaatccgtggttttacaaccctgaagtttgataatagctctcttggatttttgtggttacctcatggcaatctcactaagaagcaggggagcaagctcttggcacatgaaggaataggctcatgaagattcatttcttttcccgcttggccttttggttctctaataagctgtgagctgaggtccatgcagggaaaacaaggagggtaacggcaaatgtaaagtgaatttttctggagaaggatgctgattattttatagcatctacactatcctatgatgaaagaggcatagagccgggtggcaatgtgagttcttgggtgatttaataagccatcgagtggatttaatttctaagtaagacatttgtttattctttgtacaagtccatggagttgtgatcttaaagagttctgtgttatttgcattgtgcctcatttctccccatcaaccttagcttgagatttggatgaataaaataaataactggagaaggttaaagtatgcaccaa

SEQ ID NO: 36 - RNA, 25 nt, synthetic construct
  source 1..25: mol_type = other RNA
cagtaaatcagatagtagccttgaa

SEQ ID NO: 37 - RNA, 25 nt, synthetic construct
  source 1..25: mol_type = other RNA
gtctaatataagttggaagctgtac

SEQ ID NO: 38 - RNA, 25 nt, synthetic construct
  source 1..25: mol_type = other RNA
gatccattcaatgatctcaccgagg

SEQ ID NO: 39 - RNA, 25 nt, synthetic construct
  source 1..25: mol_type = other RNA
tatgtgtgcatttctgaggccactt

SEQ ID NO: 40 - RNA, 25 nt, synthetic construct
  source 1..25: mol_type = other RNA
atgaatgtttattcccattcccaaa

SEQ ID NO: 41 - RNA, 25 nt, synthetic construct
  source 1..25: mol_type = other RNA
ctcccaactcccaaggctacccaag

SEQ ID NO: 42 - RNA, 25 nt, synthetic construct
  source 1..25: mol_type = other RNA
aaggactccatttccagtgcagaag

SEQ ID NO: 43 - RNA, 25 nt, synthetic construct
  source 1..25: mol_type = other RNA
aatgcaagtgctgggagggaccaag

SEQ ID NO: 44 - RNA, 25 nt, synthetic construct
  source 1..25: mol_type = other RNA
accgtatgtctgtgtaccacccatc

SEQ ID NO: 45 - RNA, 25 nt, synthetic construct
  source 1..25: mol_type = other RNA
tacgtgtcactctgacagctccata

SEQ ID NO: 46 - RNA, 25 nt, synthetic construct
  source 1..25: mol_type = other RNA
atgagtatagctggataaggcctcc

SEQ ID NO: 47 - RNA, 25 nt, synthetic construct
  source 1..25: mol_type = other RNA
attaatgtcatagggaggaaagttg

SEQ ID NO: 48 - RNA, 25 nt, synthetic construct
  source 1..25: mol_type = other RNA
ctgctagagctttagacactgcatt

SEQ ID NO: 49 - RNA, 25 nt, synthetic construct
  source 1..25: mol_type = other RNA
ctcgattgagcagtgagtacacaaa

SEQ ID NO: 50 - RNA, 25 nt, synthetic construct
  source 1..25: mol_type = other RNA
tggataactggttagcagtgctatg

SEQ ID NO: 51 - RNA, 25 nt, synthetic construct
  source 1..25: mol_type = other RNA
aaagatgaatggaataagggctttc

SEQ ID NO: 52 - RNA, 25 nt, synthetic construct
  source 1..25: mol_type = other RNA
tggtgaaaagctcgcagcccaagga

SEQ ID NO: 53 - RNA, 25 nt, synthetic construct
  source 1..25: mol_type = other RNA
agtaatgtaggcagaagaggcccag

SEQ ID NO: 54 - RNA, 25 nt, synthetic construct
  source 1..25: mol_type = other RNA
ccagaaacatacgtaaacaagccac

SEQ ID NO: 55 - RNA, 25 nt, synthetic construct
  source 1..25: mol_type = other RNA
caccgcgaaggaaggcagctcctgc

SEQ ID NO: 56 - RNA, 25 nt, synthetic construct
  source 1..25: mol_type = other RNA
cttcaggctctccgtgtgcttcccg

SEQ ID NO: 57 - RNA, 25 nt, synthetic construct
  source 1..25: mol_type = other RNA
gcgacgtacaaggccagtgccccaa

SEQ ID NO: 58 - DNA, 4828 bp, synthetic construct
  source 1..4828: mol_type = other DNA
cctgcaggcagctgcgcgctcgctcgctcactgaggccgcccgggcgtcgggcgacctttggtcgcccggcctcagtgagcgagcgagcgcgcagagagggagtggccaactccatcactaggggttcctgcggcctctagactcgaggcgttgacattgattattgactagttattaatagtaatcaattacggggtcattagttcatagcccatatatggagttccgcgttacataacttacggtaaatggcccgcctggctgaccgcccaacgacccccgcccattgacgtcaataatgacgtatgttcccatagtaacgccaatagggactttccattgacgtcaatgggtggagtatttacggtaaactgcccacttggcagtacatcaagtgtatcatatgccaagtacgccccctattgacgtcaatgacggtaaatggcccgcctggcattatgcccagtacatgaccttatgggactttcctacttggcagtacatctacgtattagtcatcgctattaccatggtgatgcggttttggcagtacatcaatgggcgtggatagcggtttgactcacggggatttccaagtctccaccccattgacgtcaatgggagtttgttttggcaccaaaatcaacgggactttccaaaatgtcgtaacaactccgccccattgacgcaaatgggcggtaggcgtgtacggtgggaggtctatataagcagagctctctggctaactaccggtgccaccatggtgagcaagggcgaggagctgttcaccggggtggtgcccatcctggtcgagctggacggcgacgtaaacggccacaagttcagcgtgtccggcgagggcgagggcgatgccacctacggcaagctgaccctgaagttcatctgcaccaccggcaagctgcccgtgccctggcccaccctcgtgaccaccctgacctacggcgtgcagtgcttcagccgctaccccgaccacatgaagcagcacgacttcttcaagtccgccatgcccgaaggctacgtccaggagcgcaccatcttcttcaaggacgacggcaactacaagacccgcgccgaggtgaagttcgagggcgacaccctggtgaaccgcatcgagctgaagggcatcgacttcaaggaggacggcaacatcctggggcacaagctggagtacaactacaacagccacaacgtctatatcatggccgacaagcagaagaacggcatcaaggtgaacttcaagatccgccacaacatcgaggacggcagcgtgcagctcgccgaccactaccagcagaacacccccatcggcgacggccccgtgctgctgcccgacaaccactacctgagcacccagtccgccctgagcaaagaccccaacgagaagcgcgatcacatggtcctgctggagttcgtgaccgccgccgggatcactctcggcatggacgagctgtacaagtaaagcggccgaattcctagagctcgctgatcagcctcgactgtgccttctagttgccagccatctgttgtttgcccctcccccgtgccttccttgaccctggaaggtgccactcccactgtcctttcctaataaaatgaggaaattgcatcgcattgtctgagtaggtgtcattctattctggggggtggggtggggcaggacagcaagggggaggattgggaagagaatagcaggcatgctggggaggtaccgagggcctatttcccatgattccttcatatttgcatatacgatacaaggctgttagagagataattggaattaatttgactgtaaacacaaagatattagtacaaaatacgtgacgtagaaagtaataatttcttgggtagtttgcagttttaaaattatgttttaaaatggactatcatatgcttaccgtaacttgaaagtatttcgatttcttggctttatatatcttgtggaaaggacgaaacaccggagaccacggcaggtctcagttttagtactctggaaacagaatctactaaaacaaggcaaaatgccgtgtttatctcgtcaacttgttggcgagatttttgcggccgcaggaacccctagtgatggagttggccactccctctctgcgcgctcgctcgctcactgaggccgggcgaccaaaggtcgcccgacgcccgggctttgcccgggcggcctcagtgagcgagcgagcgcgcagctgcctgcaggggcgcctgatgcggtattttctccttacgcatctgtgcggtatttcacaccgcatacgtcaaagcaaccatagtacgcgccctgtagcggcgcattaagcgcggcgggtgtggtggttacgcgcagcgtgaccgctacacttgccagcgccctagcgcccgctcctttcgctttcttcccttcctttctcgccacgttcgccggctttccccgtcaagctctaaatcgggggctccctttagggttccgatttagtgctttacggcacctcgaccccaaaaaacttgatttgggtgatggttcacgtagtgggccatcgccctgatagacggtttttcgccctttgacgttggagtccacgttctttaatagtggactcttgttccaaactggaacaacactcaaccctatctcgggctattcttttgatttataagggattttgccgatttcggcctattggttaaaaaatgagctgatttaacaaaaatttaacgcgaattttaacaaaatattaacgtttacaattttatggtgcactctcagtacaatctgctctgatgccgcatagttaagccagccccgacacccgccaacacccgctgacgcgccctgacgggcttgtctgctcccggcatccgcttacagacaagctgtgaccgtctccgggagctgcatgtgtcagaggttttcaccgtcatcaccgaaacgcgcgagacgaaagggcctcgtgatacgcctatttttataggttaatgtcatgataataatggtttcttagacgtcaggtggcacttttcggggaaatgtgcgcggaacccctatttgtttatttttctaaatacattcaaatatgtatccgctcatgagacaataaccctgataaatgcttcaataatattgaaaaaggaagagtatgagtattcaacatttccgtgtcgcccttattcccttttttgcggcattttgccttcctgtttttgctcacccagaaacgctggtgaaagtaaaagatgctgaagatcagttgggtgcacgagtgggttacatcgaactggatctcaacagcggtaagatccttgagagttttcgccccgaagaacgttttccaatgatgagcacttttaaagttctgctatgtggcgcggtattatcccgtattgacgccgggcaagagcaactcggtcgccgcatacactattctcagaatgacttggttgagtactcaccagtcacagaaaagcatcttacggatggcatgacagtaagagaattatgcagtgctgccataaccatgagtgataacactgcggccaacttacttctgacaacgatcggaggaccgaaggagctaaccgcttttttgcacaacatgggggatcatgtaactcgccttgatcgttgggaaccggagctgaatgaagccataccaaacgacgagcgtgacaccacgatgcctgtagcaatggcaacaacgttgcgcaaactattaactggcgaactacttactctagcttcccggcaacaattaatagactggatggaggcggataaagttgcaggaccacttctgcgctcggcccttccggctggctggtttattgctgataaatctggagccggtgagcgtggaagccgcggtatcattgcagcactggggccagatggtaagccctcccgtatcgtagttatctacacgacggggagtcaggcaactatggatgaacgaaatagacagatcgctgagataggtgcctcactgattaagcattggtaactgtcagaccaagtttactcatatatactttagattgatttaaaacttcatttttaatttaaaaggatctaggtgaagatcctttttgataatctcatgaccaaaatcccttaacgtgagttttcgttccactgagcgtcagaccccgtagaaaagatcaaaggatcttcttgagatcctttttttctgcgcgtaatctgctgcttgcaaacaaaaaaaccaccgctaccagcggtggtttgtttgccggatcaagagctaccaactctttttccgaaggtaactggcttcagcagagcgcagataccaaatactgtccttctagtgtagccgtagttaggccaccacttcaagaactctgtagcaccgcctacatacctcgctctgctaatcctgttaccagtggctgctgccagtggcgataagtcgtgtcttaccgggttggactcaagacgatagttaccggataaggcgcagcggtcgggctgaacggggggttcgtgcacacagcccagcttggagcgaacgacctacaccgaactgagatacctacagcgtgagctatgagaaagcgccacgcttcccgaagggagaaaggcggacaggtatccggtaagcggcagggtcggaacaggagagcgcacgagggagcttccagggggaaacgcctggtatctttatagtcctgtcgggtttcgccacctctgacttgagcgtcgatttttgtgatgctcgtcaggggggcggagcctatggaaaaacgccagcaacgcggcctttttacggttcctggccttttgctggccttttgctcacatgt

SEQ ID NO: 59 - RNA, 21 nt, synthetic construct
  source 1..21: mol_type = other RNA
ggaggccttatccagctatac

SEQ ID NO: 60 - RNA, 21 nt, synthetic construct
  source 1..21: mol_type = other RNA
gggaatgggaataaacattca

SEQ ID NO: 61 - DNA, 59 bp, synthetic construct
  source 1..59: mol_type = other DNA
caccgggaggccttatccagctatacctcgaggtatagctggataaggcctcctttttt

SEQ ID NO: 62 - DNA, 59 bp, synthetic construct
  source 1..59: mol_type = other DNA
ggccaaaaaaggaggccttatccagctatacctcgaggtatagctggataaggcctccc

SEQ ID NO: 63 - DNA, 59 bp, synthetic construct
  source 1..59: mol_type = other DNA
caccggggaatgggaataaacattcactcgagtgaatgtttattcccattccctttttt

SEQ ID NO: 64 - DNA, 59 bp, synthetic construct
  source 1..59: mol_type = other DNA
ggccaaaaaagggaatgggaataaacattcactcgagtgaatgtttattcccattcccc

SEQ ID NO: 65 - DNA, 9285 bp, synthetic construct
  source 1..9285: mol_type = other DNA
gtcgacggatcgggagatctcccgatcccctatggtgcactctcagtacaatctgctctgatgccgcatagttaagccagtatctgctccctgcttgtgtgttggaggtcgctgagtagtgcgcgagcaaaatttaagctacaacaaggcaaggcttgaccgacaattgcatgaagaatctgcttagggttaggcgttttgcgctgcttcgcgatgtacgggccagatatacgcgttgacattgattattgactagttattaatagtaatcaattacggggtcattagttcatagcccatatatggagttccgcgttacataacttacggtaaatggcccgcctggctgaccgcccaacgacccccgcccattgacgtcaataatgacgtatgttcccatagtaacgccaatagggactttccattgacgtcaatgggtggagtatttacggtaaactgcccacttggcagtacatcaagtgtatcatatgccaagtacgccccctattgacgtcaatgacggtaaatggcccgcctggcattatgcccagtacatgaccttatgggactttcctacttggcagtacatctacgtattagtcatcgctattaccatggtgatgcggttttggcagtacatcaatgggcgtggatagcggtttgactcacggggatttccaagtctccaccccattgacgtcaatgggagtttgttttggcaccaaaatcaacgggactttccaaaatgtcgtaacaactccgccccattgacgcaaatgggcggtaggcgtgtacggtgggaggtctatagaccagatctgagcctgggagctctctggctaactagggaacccactgcttaagcctcaataaagcttgccttgagtgcttcaagtagtgtgtgcccgtctgttgtgtgactctggtaactagagatccctcagacccttttagtcagtgtggaaaatctctagcagtggcgcccgaacagggacttgaaagcgaaagggaaaccagaggagctctctcgacgcaggactcggcttgctgaagcgcgcacggcaagaggcgaggggcggcgactggtgagtacgccaaaaattttgactagcggaggctagaaggagagagatgggtgcgagagcgtcagtattaagcgggggagaattagatcgcgatgggaaaaaattcggttaaggccagggggaaagaaaaaatataaataaacatatagtatgggcaagcagggagctagaacgattcgcagttaatcctggcctgttagaaacatcagaaggctgtagacaaatactgggacagctacaaccatcccttcagacaggatcagaagaacttagatcattatataatacagtagcaaccctctattgtgtgcatcaaaggatagagataaaagacaccaaggaagctttagacaagatagaggaagagcaaaacaaaagtaagaccaccgcacagcaagcggccggccgcgctgatcttcagacctggaggaggagatatgagggacaattggagaagtgaattatataaatataaagtagtaaaaattgaaccattaggagtagcacccaccaaggcaaagagaagagtggtgcagagagaaaaaagagcagtgggaataggagctttgttccttgggttcttgggagcagcaggaagcactatgggcgcagcgtcaatgacgctgacggtacaggccagacaattattgtctggtatagtgcagcagcagaacaatttgctgagggctattgaggcgcaacagcatctgttgcaactcacagtctggggcatcaagcagctccaggcaagaatcctggctgtggaaagatacctaaaggatcaacagctcctggggatttggggttgctctggaaaactcatttgcaccactgctgtgccttggaatgctagttggagtaataaatctctggaacagatttggaatcacacgacctggatggagtgggacagagaaattaacaattacacaagcttaatacactccttaattgaagaatcgcaaaaccagcaagaaaagaatgaacaagaattattggaattagataaatgggcaagtttgtggaattggtttaacataacaaattggctgtggtatataaaattattcataatgatagtaggaggcttggtaggtttaagaatagtttttgctgtactttctatagtgaatagagttaggcagggatattcaccattatcgtttcagacccacctcccaaccccgaggggacccgacaggcccgaaggaatagaagaagaaggtggagagagagacagagacagatccattcgattagtgaacggatcggcactgcgtgcgccaattctgcagacaaatggcagtattcatccacaattttaaaagaaaaggggggattggggggtacagtgcaggggaaagaatagtagacataatagcaacagacatacaaactaaagaattacaaaaacaaattacaaaaattcaaaattttcgggtttattacagggacagcagagatccagtttggttagtaccgggcccgctctagcgtcgaggagcttggcccattgcatacgttgtatccatatcataatatgtacatttatattggctcatgtccaacattaccgccatgttgacattgattattgactagttattaatagtaatcaattacggggtcattagttcatagcccatatatggagttccgcgttacataacttacggtaaatggcccgcctggctgaccgcccaacgacccccgcccattgacgtcaataatgacgtatgttcccatagtaacgccaatagggactttccattgacgtcaatgggtggagtatttacggtaaactgcccacttggcagtacatcaagtgtatcatatgccaagtacgccccctattgacgtcaatgacggtaaatggcccgcctggcattatgcccagtacatgaccttatgggactttcctacttggcagtacatctacgtattagtcatcgctattaccatggtgatgcggttttggcagtacatcaatgggcgtggatagcggtttgactcacggggatttccaagtctccaccccattgacgtcaatgggagtttgttttggcaccaaaatcaacgggactttccaaaatgtcgtaacaactccgccccattgacgcaaatgggcggtaggcgtgtacggtgggaggtctatataagcagagctcgtttagtgaaccgtcagatcgcctggagacgccatccacgctgttttgacctccatagaagacaccgggaccgatccagcctccgcggccccgaattcgccaccatgcaggttcagtgccagcagagcccagtgctggcaggcagcgccactttggtcgcccttggggcactggccttgtacgtcgcgaagccctccggctacgggaagcacacggagagcctgaagccggcggctacccgcctgccagcccgcgccgcctggttcctgcaggagctgccttccttcgcggtgcccgcggggatcctcgcccggcagcccctctccctcttcgggccacctgggacggtacttctgggcctcttctgcctacattacttccacaggacatttgtgtactcactgctcaatcgagggaggccttatccagctatactcattctcagaggcactgccttctgcactggaaatggagtccttcaaggctactatctgatttactgtgctgaataccctgatgggtggtacacagacatacggtttagcttgggtgtcttcttatttattttgggaatgggaataaacattcatagtgactatatattgcgccagctcaggaagcctggagaaatcagctacaggattccacaaggtggcttgtttacgtatgtttctggagccaatttcctcggtgagatcattgaatggatcggctatgccctggccacttggtccctcccagcacttgcatttgcatttttctcactttgtttccttgggctgcgagcttttcaccaccataggttctacctcaagatgtttgaggactaccccaaatctcggaaagcccttattccattcatctttgctagcggcagtggagagggcagaggaagtctgctaacatgcggtgacgtcgaggagaatcctggcccagtgagcaagggcgaggagctgttcaccggggtggtgcccatcctggtcgagctggacggcgacgtaaacggccacaagttcagcgtgtccggcgagggcgagggcgatgccacctacggcaagctgaccctgaagttcatctgcaccaccggcaagctgcccgtgccctggcccaccctcgtgaccaccctgacctacggcgtgcagtgcttcagccgctaccccgaccacatgaagcagcacgacttcttcaagtccgccatgcccgaaggctacgtccaggagcgcaccatcttcttcaaggacgacggcaactacaagacccgcgccgaggtgaagttcgagggcgacaccctggtgaaccgcatcgagctgaagggcatcgacttcaaggaggacggcaacatcctggggcacaagctggagtacaactacaacagccacaacgtctatatcatggccgacaagcagaagaacggcatcaaggtgaacttcaagatccgccacaacatcgaggacggcagcgtgcagctcgccgaccactaccagcagaacacccccatcggcgacggccccgtgctgctgcccgacaaccactacctgagcacccagtccgccctgagcaaagaccccaacgagaagcgcgatcacatggtcctgctggagttcgtgaccgccgccgggatcactctcggcatggacgagctgtacaagtaaggatcctaggcggccgcgcatgccctgcaggtgatctatcgatcggccggcccctctccctccccccccccctaacgttactggccgaagccgcttggaataaggccggtgtgcgtttgtctatatgttattttccaccatattgccgtcttttggcaatgtgagggcccggaaacctggccctgtcttcttgacgagcattcctaggggtctttcccctctcgccaaaggaatgcaaggtctgttgaatgtcgtgaaggaagcagttcctctggaagcttcttgaagacaaacaacgtctgtagcgaccctttgcaggcagcggaaccccccacctggcgacaggtgcctctgcggccaaaagccacgtgtataagatacacctgcaaaggcggcacaaccccagtgccacgttgtgagttggatagttgtggaaagagtcaaatggctctcctcaagcgtattcaacaaggggctgaaggatgcccagaaggtaccccattgtatgggatctgatctggggcctcggtacacatgctttacatgtgtttagtcgaggttaaaaaaacgtctaggccccccgaaccacggggacgtggttttcctttgaaaaacacgatgataatatggccacaaccgggccggatatcacgcgtgatctgatcagcacgtgttgacaattaatcatcggcatagtatatcggcatagtataatacgacaaggtgaggaactaaaccatggccaagcctttgtctcaagaagaatccaccctcattgaaagagcaacggctacaatcaacagcatccccatctctgaagactacagcgtcgccagcgcagctctctctagcgacggccgcatcttcactggtgtcaatgtatatcattttactgggggaccttgtgcagaactcgtggtgctgggcactgctgctgctgcggcagctggcaacctgacttgtatcgtcgcgatcggaaatgagaacaggggcatcttgagcccctgcggacggtgccgacaggtgcttctcgatctgcatcctgggatcaaagccatagtgaaggacagtgatggacagccgacggcagttgggattcgtgaattgctgccctctggttatgtgtgggagggctaagcaatgcatacatgtgtttaaacctcgacttaattaagtcgagggtcgacggtatcgataagctcgcttcacgagatcatgtttaagggttccggttccactaggtacaattcgatatcaagcttatcgataatcaacctctggattacaaaatttgtgaaagattgactggtattcttaactatgttgctccttttacgctatgtggatacgctgctttaatgcctttgtatcatgctattgcttcccgtatggctttcattttctcctccttgtataaatcctggttgctgtctctttatgaggagttgtggcccgttgtcaggcaacgtggcgtggtgtgcactgtgtttgctgacgcaacccccactggttggggcattgccaccacctgtcagctcctttccgggactttcgctttccccctccctattgccacggcggaactcatcgccgcctgccttgcccgctgctggacaggggctcggctgttgggcactgacaattccgtggtgttgtcggggaaatcatcgtcctttccttggctgctcgcctgtgttgccacctggattctgcgcgggacgtccttctgctacgtcccttcggccctcaatccagcggaccttccttcccgcggcctgctgccggctctgcggcctcttccgcgtcttcgccttcgccctcagacgagtcggatctccctttgggccgcctccccgcatcgataccgtcgacctcgatcgagacctagaaaaacatggagcaatcacaagtagcaatacagcagctaccaatgctgattgtgcctggctagaagcacaagaggaggaggaggtgggttttccagtcacacctcaggtacctttaagaccaatgacttacaaggcagctgtagatcttagccactttttaaaagaaaaggggggactggaagggctaattcactcccaacgaagacaagatatccttgatctgtggatctaccacacacaaggctacttccctgattggcagaactacacaccagggccagggatcagatatccactgacctttggatggtgctacaagctagtaccagttgagcaagagaaggtagaagaagccaatgaaggagagaacacccgcttgttacaccctgtgagcctgcatgggatggatgacccggagagagaagtattagagtggaggtttgacagccgcctagcatttcatcacatggcccgagagctgcatccggactgtactgggtctctctggttagaccagatctgagcctgggagctctctggctaactagggaacccactgcttaagcctcaataaagcttgccttgagtgcttcaagtagtgtgtgcccgtctgttgtgtgactctggtaactagagatccctcagacccttttagtcagtgtggaaaatctctagcagcatgtgagcaaaaggccagcaaaaggccaggaaccgtaaaaaggccgcgttgctggcgtttttccataggctccgcccccctgacgagcatcacaaaaatcgacgctcaagtcagaggtggcgaaacccgacaggactataaagataccaggcgtttccccctggaagctccctcgtgcgctctcctgttccgaccctgccgcttaccggatacctgtccgcctttctcccttcgggaagcgtggcgctttctcatagctcacgctgtaggtatctcagttcggtgtaggtcgttcgctccaagctgggctgtgtgcacgaaccccccgttcagcccgaccgctgcgccttatccggtaactatcgtcttgagtccaacccggtaagacacgacttatcgccactggcagcagccactggtaacaggattagcagagcgaggtatgtaggcggtgctacagagttcttgaagtggtggcctaactacggctacactagaagaacagtatttggtatctgcgctctgctgaagccagttaccttcggaaaaagagttggtagctcttgatccggcaaacaaaccaccgctggtagcggtggtttttttgtttgcaagcagcagattacgcgcagaaaaaaaggatctcaagaagatcctttgatcttttctacggggtctgacgctcagtggaacgaaaactcacgttaagggattttggtcatgagattatcaaaaaggatcttcacctagatccttttaaattaaaaatgaagttttaaatcaatctaaagtatatatgagtaaacttggtctgacagttaccaatgcttaatcagtgaggcacctatctcagcgatctgtctatttcgttcatccatagttgcctgactccccgtcgtgtagataactacgatacgggagggcttaccatctggccccagtgctgcaatgataccgcgagacccacgctcaccggctccagatttatcagcaataaaccagccagccggaagggccgagcgcagaagtggtcctgcaactttatccgcctccatccagtctattaattgttgccgggaagctagagtaagtagttcgccagttaatagtttgcgcaacgttgttgccattgctacaggcatcgtggtgtcacgctcgtcgtttggtatggcttcattcagctccggttcccaacgatcaaggcgagttacatgatcccccatgttgtgcaaaaaagcggttagctccttcggtcctccgatcgttgtcagaagtaagttggccgcagtgttatcactcatggttatggcagcactgcataattctcttactgtcatgccatccgtaagatgcttttctgtgactggtgagtactcaaccaagtcattctgagaatagtgtatgcggcgaccgagttgctcttgcccggcgtcaatacgggataataccgcgccacatagcagaactttaaaagtgctcatcattggaaaacgttcttcggggcgaaaactctcaaggatcttaccgctgttgagatccagttcgatgtaacccactcgtgcacccaactgatcttcagcatcttttactttcaccagcgtttctgggtgagcaaaaacaggaaggcaaaatgccgcaaaaaagggaataagggcgacacggaaatgttgaatactcatactcttcctttttcaatattattgaagcatttatcagggttattgtctcatgagcggatacatatttgaatgtatttagaaaaataaacaaataggggttccgcgcacatttccccgaaaagtgccacctgac

SEQ ID NO: 66 - DNA, 19 bp, synthetic construct
  source 1..19: mol_type = other DNA
actgctcaatcgagggagg

SEQ ID NO: 67 - DNA, 22 bp, synthetic construct
  source 1..22: mol_type = other DNA
cacccaagctaaaccgtatgtc

SEQ ID NO: 68 - DNA, 21 bp, synthetic construct
  source 1..21: mol_type = other DNA
cggtttagcttgggtgtcttc

SEQ ID NO: 69 - DNA, 21 bp, synthetic construct
  source 1..21: mol_type = other DNA
ccgaggaaattggctccagaa

SEQ ID NO: 70 - DNA, 7013 bp, synthetic construct
  source 1..7013: mol_type = other DNA
cctgcaggcagctgcgcgctcgctcgctcactgaggccgcccgggcgtcgggcgacctttggtcgcccggcctcagtgagcgagcgagcgcgcagagagggagtggccaactccatcactaggggttcctgcggcctctagactcgaggcgttgacattgattattgactagttattaatagtaatcaattacggggtcattagttcatagcccatatatggagttccgcgttacataacttacggtaaatggcccgcctggctgaccgcccaacgacccccgcccattgacgtcaataatgacgtatgttcccatagtaacgccaatagggactttccattgacgtcaatgggtggagtatttacggtaaactgcccacttggcagtacatcaagtgtatcatatgccaagtacgccccctattgacgtcaatgacggtaaatggcccgcctggcattatgcccagtacatgaccttatgggactttcctacttggcagtacatctacgtattagtcatcgctattaccatggtgatgcggttttggcagtacatcaatgggcgtggatagcggtttgactcacggggatttccaagtctccaccccattgacgtcaatgggagtttgttttggcaccaaaatcaacgggactttccaaaatgtcgtaacaactccgccccattgacgcaaatgggcggtaggcgtgtacggtgggaggtctatataagcagagctctctggctaactaccggtgccaccatgccggcagctaagaaaaagaaactggatggcagcgtcgacatcgagaagaaaaaatcctttgctaagggcatgggcgttaagagcactctggtgtcaggctctaaagtgtacatgaccacattcgccgagggctctgatgctcgcctggaaaaaattgtggaaggagactcaatcagatccgtgaacgagggggaggccttcagcgccgagatggccgacaagaatgccggatataagattggaaacgctaagttcagccatcccaagggatacgccgtggtcgccaacaatcctctgtacactggacctgtgcagcaggacatgttaggtctgaaggagactctggagaagaggtacttcggcgagtccgcagatggcaacgacaacatttgcattcaggtgatccataacatcctggacattgagaagatcctggccgagtatatcaccaacgcagcctacgctgtgaataatatatctggtctggataaggatatcattgggttcgggaaattttctaccgtgtacacctacgatgagtttaaagaccccgagcaccacagagccgccttcaacaacaacgacaagctgatcaatgccattaaggcacagtacgatgagttcgacaattttctggacaacccccggctgggctacttcggccaggcttttttttctaaggaaggccgcaattacatcatcaactacggcaacgagtgctatgacattctggcccttctgagcggcctgaggcattgggtggtgcataacaacgaagaggaatcccgcatctcaagaacatggctgtacaatctcgacaaaaacctggacaatgagtacatttccactctgaactatctgtacgacaggatcacgaatgagctgaccaattccttttccaagaatagcgccgccaatgtgaactacatcgccgaaaccctggggatcaatcccgccgagttcgccgagcagtattttcgattcagcatcatgaaagagcagaaaaatctgggctttaatatcaccaaactgagagaagtgatgctggacaggaaggatatgtctgagatcaggaagaaccacaaggtgttcgacagtatcagaaccaaggtgtatacaatgatggatttcgtgatctataggtactacattgaggaggacgccaaggtggccgccgccaacaaatccctgcctgataacgagaagtccctgtctgagaaggatatcttcgtcatcaacctgaggggcagcttcaatgatgaccagaaggacgctctttactacgacgaagccaaccggatctggcggaagctggaaaacatcatgcacaacatcaaggagttccgcgggaacaaaacacgggagtacaagaaaaaagacgctcccagactgcccagaatcctgcctgcaggcagggatgtgagcgcattctccaagctgatgtacgccctgacaatgttcctggatggcaaggaaatcaacgacctgctgaccactctgatcaacaagtttgataacattcagagctttctgaaagtgatgcccctgatcggagtgaatgcaaaattcgtcgaagaatacgctttcttcaaggattctgctaaaatcgccgacgagctgaggctgattaagtcctttgcaaggatgggggagccaatcgccgacgccagaagagccatgtatattgatgctatcagaatcctgggcaccaatctgtcctatgacgaactgaaggccctggctgacacattttctctggatgagaatggtaacaagctgaagaaggggaagcacggcatgcgaaactttattattaacaatgttatctctaataagaggttccattatctgattcgctacggcgaccccgcccatttgcacgagatcgccaagaatgaagcggtggtgaagttcgtcctgggacggatcgccgacatccagaaaaagcagggccagaatggcaaaaaccagatcgacagatattatgagacttgcatcggcaaggataagggtaaaagtgtctccgagaaagtggatgccctgactaagatcattacggggatgaattacgaccagtttgacaaaaagaggagcgtgatcgaggacaccggcagagagaatgccgagcgggagaagtttaagaagatcatcagcctgtatctgaccgtgatttaccatatcctgaagaatatcgtgaatatcaatgccagatacgtgatcggcttccactgcgtggaaagagacgcccagctctacaaagagaaaggctacgacatcaatctgaagaagctggaggaaaagggctttagcagcgtgacaaaactgtgtgcaggaatcgacgagactgcccctgacaagaggaaggacgtggagaaagagatggccgaacgcgccaaggagtctatcgactccctggagtccgccaaccccaagctgtacgccaactacatcaagtatagcgacgagaagaaggcagaagagttcacccggcagatcaatagagagaaggccaaaaccgcactgaatgcctatctgaggaatacaaagtggaacgtgattattagagaagatctgctgaggattgacaataagacctgtaccctattcaggaacaaggccgtgcatctggaggtggccaggtacgtgcatgcctatattaatgatatagctgaagtcaactcctatttccagctgtatcattacatcatgcagcgtattattatgaacgaaagatatgaaaagagctccggcaaagtgtctgagtacttcgatgccgtgaacgacgaaaaaaagtacaatgatcgcctgctgaagctgctgtgtgtgcccttcgggtactgtatccccagatttaagaatctgtccattgaagccctgttcgatagaaacgaagccgccaaattcgacaaggagaagaagaaggtgagcggcaatagtacaggcggcggccccggcggcggcgccgccgccggcagcggcagccctaagaaaaaacgaaaagttggcagcggaagcaaaaggccggcggccacgaaaaaggccggccaggcaaaaaagaaaaagctcgagtacccatacgatgttccagattacgcttgagaattccccttgagcatctgacttctggctaataaaggaaatttattttcattgcaatagtgtgttggaattttttgtgtctctcaggtaccgagggcctatttcccatgattccttcatatttgcatatacgatacaaggctgttagagagataattggaattaatttgactgtaaacacaaagatattagtacaaaatacgtgacgtagaaagtaataatttcttgggtagtttgcagttttaaaattatgttttaaaatggactatcatatgcttaccgtaacttgaaagtatttcgatttcttggctttatatatcttgtggaaaggacgaaacaccgcaagtaaacccctaccaactggtcggggtttgaaacggagaccacggcaggtctcattttttgcggccgcaggaacccctagtgatggagttggccactccctctctgcgcgctcgctcgctcactgaggccgggcgaccaaaggtcgcccgacgcccgggctttgcccgggcggcctcagtgagcgagcgagcgcgcagctgcctgcaggggcgcctgatgcggtattttctccttacgcatctgtgcggtatttcacaccgcatacgtcaaagcaaccatagtacgcgccctgtagcggcgcattaagcgcggcgggtgtggtggttacgcgcagcgtgaccgctacacttgccagcgccttagcgcccgctcctttcgctttcttcccttcctttctcgccacgttcgccggctttccccgtcaagctctaaatcgggggctccctttagggttccgatttagtgctttacggcacctcgaccccaaaaaacttgatttgggtgatggttcacgtagtgggccatcgccctgatagacggtttttcgccctttgacgttggagtccacgttctttaatagtggactcttgttccaaactggaacaacactcaactctatctcgggctattcttttgatttataagggattttgccgatttcggtctattggttaaaaaatgagctgatttaacaaaaatttaacgcgaattttaacaaaatattaacgtttacaattttatggtgcactctcagtacaatctgctctgatgccgcatagttaagccagccccgacacccgccaacacccgctgacgcgccctgacgggcttgtctgctcccggcatccgcttacagacaagctgtgaccgtctccgggagctgcatgtgtcagaggttttcaccgtcatcaccgaaacgcgcgagacgaaagggcctcgtgatacgcctatttttataggttaatgtcatgataataatggtttcttagacgtcaggtggcacttttcggggaaatgtgcgcggaacccctatttgtttatttttctaaatacattcaaatatgtatccgctcatgagacaataaccctgataaatgcttcaataatattgaaaaaggaagagtatgagtattcaacatttccgtgtcgcccttattcccttttttgcggcattttgccttcctgtttttgctcacccagaaacgctggtgaaagtaaaagatgctgaagatcagttgggtgcacgagtgggttacatcgaactggatctcaacagcggtaagatccttgagagttttcgccccgaagaacgttttccaatgatgagcacttttaaagttctgctatgtggcgcggtattatcccgtattgacgccgggcaagagcaactcggtcgccgcatacactattctcagaatgacttggttgagtactcaccagtcacagaaaagcatcttacggatggcatgacagtaagagaattatgcagtgctgccataaccatgagtgataacactgcggccaacttacttctgacaacgatcggaggaccgaaggagctaaccgcttttttgcacaacatgggggatcatgtaactcgccttgatcgttgggaaccggagctgaatgaagccataccaaacgacgagcgtgacaccacgatgcctgtagcaatggcaacaacgttgcgcaaactattaactggcgaactacttactctagcttcccggcaacaattaatagactggatggaggcggataaagttgcaggaccacttctgcgctcggcccttccggctggctggtttattgctgataaatctggagccggtgagcgtggaagccgcggtatcattgcagcactggggccagatggtaagccctcccgtatcgtagttatctacacgacggggagtcaggcaactatggatgaacgaaatagacagatcgctgagataggtgcctcactgattaagcattggtaactgtcagaccaagtttactcatatatactttagattgatttaaaacttcatttttaatttaaaaggatctaggtgaagatcctttttgataatctcatgaccaaaatcccttaacgtgagttttcgttccactgagcgtcagaccccgtagaaaagatcaaaggatcttcttgagatcctttttttctgcgcgtaatctgctgcttgcaaacaaaaaaaccaccgctaccagcggtggtttgtttgccggatcaagagctaccaactctttttccgaaggtaactggcttcagcagagcgcagataccaaatactgttcttctagtgtagccgtagttaggccaccacttcaagaactctgtagcaccgcctacatacctcgctctgctaatcctgttaccagtggctgctgccagtggcgataagtcgtgtcttaccgggttggactcaagacgatagttaccggataaggcgcagcggtcgggctgaacggggggttcgtgcacacagcccagcttggagcgaacgacctacaccgaactgagatacctacagcgtgagctatgagaaagcgccacgcttcccgaagggagaaaggcggacaggtatccggtaagcggcagggtcggaacaggagagcgcacgagggagcttccagggggaaacgcctggtatctttatagtcctgtcgggtttcgccacctctgacttgagcgtcgatttttgtgatgctcgtcaggggggcggagcctatggaaaaacgccagcaacgcggcctttttacggttcctggccttttgctggccttttgctcacatgt

SEQ ID NO: 71 - DNA, 25 bp, synthetic construct
  source 1..25: mol_type = other DNA
tgcatgcaatgatacgatcgagttc

SEQ ID NO: 72 - DNA, 25 bp, synthetic construct
  source 1..25: mol_type = other DNA
agtactgaatgacagccatctggtc

SEQ ID NO: 73 - DNA, 25 bp, synthetic construct
  source 1..25: mol_type = other DNA
ataacatttccgaagacgacaagat

SEQ ID NO: 74 - DNA, 25 bp, synthetic construct
  source 1..25: mol_type = other DNA
aagaagaccttgcagcttccacatg

SEQ ID NO: 75 - DNA, 25 bp, synthetic construct
  source 1..25: mol_type = other DNA
aggacattcagaaagatgggctgac

SEQ ID NO: 76 - DNA, 25 bp, synthetic construct
  source 1..25: mol_type = other DNA
gttcattgaggctagagagcaaggc

SEQ ID NO: 77 - DNA, 25 bp, synthetic construct
  source 1..25: mol_type = other DNA
aatgctgaagagtagcagtgctttc

SEQ ID NO: 78 - DNA, 25 bp, synthetic construct
  source 1..25: mol_type = other DNA
agagctccatagtgacacccagaag

SEQ ID NO: 79 - DNA, 25 bp, synthetic construct
  source 1..25: mol_type = other DNA
caatcatttctgctggcgcacaggt

SEQ ID NO: 80 - DNA, 25 bp, synthetic construct
  source 1..25: mol_type = other DNA
catagccttcaatgtgtgacactgt

SEQ ID NO: 81 - DNA, 25 bp, synthetic construct
  source 1..25: mol_type = other DNA
gcaaacaccatgagccccatccagg

SEQ ID NO: 82 - DNA, 25 bp, synthetic construct
  source 1..25: mol_type = other DNA
aaactcttgagagaggtgcctcatt

SEQ ID NO: 83 - DNA, 25 bp, synthetic construct
  source 1..25: mol_type = other DNA
ttgacattggtgaaggatcgccagc

SEQ ID NO: 84 - DNA, 25 bp, synthetic construct
  source 1..25: mol_type = other DNA
agcacacactacacctggctcaatg

SEQ ID NO: 85 - DNA, 25 bp, synthetic construct
  source 1..25: mol_type = other DNA
aaacatggtccctggcagtctccaa

SEQ ID NO: 86 - DNA, 30 bp, synthetic construct
  source 1..30: mol_type = other DNA
aacagattctggaaagctcctcggtaggtc

SEQ ID NO: 87 - DNA, 30 bp, synthetic construct
  source 1..30: mol_type = other DNA
gaacagattctggaaagctcctcggtaggt

SEQ ID NO: 88 - DNA, 27 bp, synthetic construct
  source 1..27: mol_type = other DNA
aacagattctggaaagctcctcggtag

SEQ ID NO: 89 - DNA, 27 bp, synthetic construct
  source 1..27: mol_type = other DNA
gaacagattctggaaagctcctcggta

SEQ ID NO: 90 - DNA, 25 bp, synthetic construct
  source 1..25: mol_type = other DNA
aacagattctggaaagctcctcggt

SEQ ID NO: 91 - DNA, 25 bp, synthetic construct
  source 1..25: mol_type = other DNA
gaacagattctggaaagctcctcgg

SEQ ID NO: 92 - DNA, 27 bp, synthetic construct
  source 1..27: mol_type = other DNA
tggatcacttcgcgcacgctctggaac

SEQ ID NO: 93 - DNA, 27 bp, synthetic construct
  source 1..27: mol_type = other DNA
tctggatcacttcgcgcacgctctgga

SEQ ID NO: 94 - DNA, 27 bp, synthetic construct
  source 1..27: mol_type = other DNA
gttctggatcacttcgcgcacgctctg

SEQ ID NO: 95 - DNA, 25 bp, synthetic construct
  source 1..25: mol_type = other DNA
tctggatcacttcgcgcacgctctg

SEQ ID NO: 96 - DNA, 25 bp, synthetic construct
  source 1..25: mol_type = other DNA
gttctggatcacttcgcgcacgctc

SEQ ID NO: 97 - DNA, 30 bp, synthetic construct
  source 1..30: mol_type = other DNA
ggatgtctttaaggtcagcggagcagctgc

SEQ ID NO: 98 - DNA, 30 bp, synthetic construct
  source 1..30: mol_type = other DNA
aggatgtctttaaggtcagcggagcagctg

SEQ ID NO: 99 - DNA, 30 bp, synthetic construct
  source 1..30: mol_type = other DNA
caggatgtctttaaggtcagcggagcagct

SEQ ID NO: 100 - DNA, 25 bp, synthetic construct
  source 1..25: mol_type = other DNA
tgtctttaaggtcagcggagcagct

SEQ ID NO: 101 - DNA, 27 bp, synthetic construct
  source 1..27: mol_type = other DNA
ggatgtctttaaggtcagcggagcagc

SEQ ID NO: 102 - DNA, 30 bp, synthetic construct
  source 1..30: mol_type = other DNA
tcaggatgtctttaaggtcagcggagcagc

SEQ ID NO: 103 - DNA, 27 bp, synthetic construct
  source 1..27: mol_type = other DNA
aggatgtctttaaggtcagcggagcag

SEQ ID NO: 104 - DNA, 30 bp, synthetic construct
  source 1..30: mol_type = other DNA
ctcaggatgtctttaaggtcagcggagcag

SEQ ID NO: 105 - DNA, 27 bp, synthetic construct
  source 1..27: mol_type = other DNA
caggatgtctttaaggtcagcggagca

SEQ ID NO: 106 - DNA, 25 bp, synthetic construct
  source 1..25: mol_type = other DNA
ggatgtctttaaggtcagcggagca

SEQ ID NO: 107 - DNA, 27 bp, synthetic construct
  source 1..27: mol_type = other DNA
tcaggatgtctttaaggtcagcggagc

SEQ ID NO: 108 - DNA, 25 bp, synthetic construct
  source 1..25: mol_type = other DNA
aggatgtctttaaggtcagcggagc

SEQ ID NO: 109 - DNA, 27 bp, synthetic construct
  source 1..27: mol_type = other DNA
ctcaggatgtctttaaggtcagcggag

SEQ ID NO: 110 - DNA, 25 bp, synthetic construct
  source 1..25: mol_type = other DNA
caggatgtctttaaggtcagcggag

SEQ ID NO: 111 - DNA, 25 bp, synthetic construct
  source 1..25: mol_type = other DNA
tcaggatgtctttaaggtcagcgga

SEQ ID NO: 112 - DNA, 25 bp, synthetic construct
  source 1..25: mol_type = other DNA
ctcaggatgtctttaaggtcagcgg

SEQ ID NO: 113 - DNA, 30 bp, synthetic construct
  source 1..30: mol_type = other DNA
taagtaattgtccttggaggaagtgggagc

SEQ ID NO: 114 - DNA, 25 bp, synthetic construct
  source 1..25: mol_type = other DNA
cgacactgccttacacaactccttg

SEQ ID NO: 115 - DNA, 27 bp, synthetic construct
  source 1..27: mol_type = other DNA
cccatggacaccgacactgccttacac

SEQ ID NO: 116 - DNA, 25 bp, synthetic construct
  source 1..25: mol_type = other DNA
cccatggacaccgacactgccttac

SEQ ID NO: 117 - DNA, 30 bp, synthetic construct
  source 1..30: mol_type = other DNA
actcagatgctccaacgcctccacacccag

SEQ ID NO: 118 - DNA, 27 bp, synthetic construct
  source 1..27: mol_type = other DNA
tcagatgctccaacgcctccacaccca

SEQ ID NO: 119 - DNA, 27 bp, synthetic construct
  source 1..27: mol_type = other DNA
ctcagatgctccaacgcctccacaccc

SEQ ID NO: 120 - DNA, 27 bp, synthetic construct
  source 1..27: mol_type = other DNA
actcagatgctccaacgcctccacacc

SEQ ID NO: 121 - DNA, 25 bp, synthetic construct
  source 1..25: mol_type = other DNA
tcagatgctccaacgcctccacacc

SEQ ID NO: 122 - DNA, 27 bp, synthetic construct
  source 1..27: mol_type = other DNA
gactcagatgctccaacgcctccacac

SEQ ID NO: 123 - DNA, 25 bp, synthetic construct
  source 1..25: mol_type = other DNA
ctcagatgctccaacgcctccacac

SEQ ID NO: 124 - DNA, 25 bp, synthetic construct
  source 1..25: mol_type = other DNA
actcagatgctccaacgcctccaca

SEQ ID NO: 125 - DNA, 25 bp, synthetic construct
  source 1..25: mol_type = other DNA
gactcagatgctccaacgcctccac

SEQ ID NO: 126 - DNA, 27 bp, synthetic construct
  source 1..27: mol_type = other DNA
agagaacctttgcattcggccaatggg

SEQ ID NO: 127 - DNA, 25 bp, synthetic construct
  source 1..25: mol_type = other DNA
agaacctttgcattcggccaatggg

SEQ ID NO: 128 - DNA, 25 bp, synthetic construct
  source 1..25: mol_type = other DNA
gagaacctttgcattcggccaatgg

SEQ ID NO: 129 - DNA, 25 bp, synthetic construct
  source 1..25: mol_type = other DNA
agagaacctttgcattcggccaatg

SEQ ID NO: 130 - DNA, 27 bp, synthetic construct
  source 1..27: mol_type = other DNA
agcagagaacctttgcattcggccaat

SEQ ID NO: 131 - DNA, 25 bp, synthetic construct
  source 1..25: mol_type = other DNA
cagttcaagtgtcccggagctccct

SEQ ID NO: 132 - DNA, 25 bp, synthetic construct
  source 1..25: mol_type = other DNA
gcagttcaagtgtcccggagctccc

SEQ ID NO: 133 - DNA, 25 bp, synthetic construct
  source 1..25: mol_type = other DNA
tagacggcagttcaagtgtcccgga

SEQ ID NO: 134 - DNA, 27 bp, synthetic construct
  source 1..27: mol_type = other DNA
agagagacagggtagacggcagttcaa

SEQ ID NO: 135 - DNA, 30 bp, synthetic construct
  source 1..30: mol_type = other DNA
aaagttgtagtagtcgcgactctggtacgc

SEQ ID NO: 136 - DNA, 30 bp, synthetic construct
  source 1..30: mol_type = other DNA
gaaagttgtagtagtcgcgactctggtacg

SEQ ID NO: 137 - DNA, 27 bp, synthetic construct
  source 1..27: mol_type = other DNA
aaagttgtagtagtcgcgactctggta

SEQ ID NO: 138 - DNA, 27 bp, synthetic construct
  source 1..27: mol_type = other DNA
gaaagttgtagtagtcgcgactctggt

SEQ ID NO: 139 - DNA, 25 bp, synthetic construct
  source 1..25: mol_type = other DNA
aaagttgtagtagtcgcgactctgg

SEQ ID NO: 140 - DNA, 27 bp, synthetic construct
  source 1..27: mol_type = other DNA
tggaaagttgtagtagtcgcgactctg

SEQ ID NO: 141 - DNA, 25 bp, synthetic construct
  source 1..25: mol_type = other DNA
gaaagttgtagtagtcgcgactctg

SEQ ID NO: 142 - DNA, 25 bp, synthetic construct
  source 1..25: mol_type = other DNA
tggaaagttgtagtagtcgcgactc

SEQ ID NO: 143 - DNA, 25 bp, synthetic construct
  source 1..25: mol_type = other DNA
cagtggaaagttgtagtagtcgcga

SEQ ID NO: 144 - DNA, 30 bp, synthetic construct
  source 1..30: mol_type = other DNA
cccaccaccaccacacggtccatacaactg

SEQ ID NO: 145 - DNA, 27 bp, synthetic construct
  source 1..27: mol_type = other DNA
ccaccaccaccacacggtccatacaac

SEQ ID NO: 146 - DNA, 27 bp, synthetic construct
  source 1..27: mol_type = other DNA
cccaccaccaccacacggtccatacaa

SEQ ID NO: 147 - DNA, 25 bp, synthetic construct
  source 1..25: mol_type = other DNA
ccaccaccaccacacggtccataca

SEQ ID NO: 148 - DNA, 25 bp, synthetic construct
  source 1..25: mol_type = other DNA
cccaccaccaccacacggtccatac

SEQ ID NO: 149 - DNA, 25 bp, synthetic construct
  source 1..25: mol_type = other DNA
gcactctgctcaccatgccgccagg

SEQ ID NO: 150 - DNA, 25 bp, synthetic construct
  source 1..25: mol_type = other DNA
ttcatctccacagatcaggcaggtc

SEQ ID NO: 151 - DNA, 27 bp, synthetic construct
  source 1..27: mol_type = other DNA
cccagaagcttcatctccacagatcag

SEQ ID NO: 152 - DNA, 30 bp, synthetic construct
  source 1..30: mol_type = other DNA
acacccagaagcttcatctccacagatcag

SEQ ID NO: 153 - DNA, 27 bp, synthetic construct
  source 1..27: mol_type = other DNA
acccagaagcttcatctccacagatca

SEQ ID NO: 154 - DNA, 25 bp, synthetic construct
  source 1..25: mol_type = other DNA
ccagaagcttcatctccacagatca

SEQ ID NO: 155 - DNA, 27 bp, synthetic construct
  source 1..27: mol_type = other DNA
acacccagaagcttcatctccacagat

SEQ ID NO: 156 - DNA, 25 bp, synthetic construct
  source 1..25: mol_type = other DNA
acccagaagcttcatctccacagat

SEQ ID NO: 157 - DNA, 27 bp, synthetic construct
  source 1..27: mol_type = other DNA
gacacccagaagcttcatctccacaga

SEQ ID NO: 158 - DNA, 25 bp, synthetic construct
  source 1..25: mol_type = other DNA
acacccagaagcttcatctccacag

SEQ ID NO: 159 - DNA, 30 bp, synthetic construct
  source 1..30: mol_type = other DNA
agagctccatagtgacacccagaagcttca

SEQ ID NO: 160 - DNA, 30 bp, synthetic construct
  source 1..30: mol_type = other DNA
gagagctccatagtgacacccagaagcttc

SEQ ID NO: 161 - DNA, 27 bp, synthetic construct
  source 1..27: mol_type = other DNA
gagctccatagtgacacccagaagctt

SEQ ID NO: 162 - DNA, 30 bp, synthetic construct
  source 1..30: mol_type = other DNA
tgagagctccatagtgacacccagaagctt

SEQ ID NO: 163 - DNA, 27 bp, synthetic construct
  source 1..27: mol_type = other DNA
agagctccatagtgacacccagaagct

SEQ ID NO: 164 - DNA, 27 bp, synthetic construct
  source 1..27: mol_type = other DNA
gagagctccatagtgacacccagaagc

SEQ ID NO: 165 - DNA, 25 bp, synthetic construct
  source 1..25: mol_type = other DNA
gagctccatagtgacacccagaagc

SEQ ID NO: 166 - DNA, 27 bp, synthetic construct
  source 1..27: mol_type = other DNA
tgagagctccatagtgacacccagaag

SEQ ID NO: 167 - DNA, 25 bp, synthetic construct
  source 1..25: mol_type = other DNA
agagctccatagtgacacccagaag

SEQ ID NO: 168 - DNA, 25 bp, synthetic construct
  source 1..25: mol_type = other DNA
gagagctccatagtgacacccagaa

SEQ ID NO: 169 - DNA, 25 bp, synthetic construct
  source 1..25: mol_type = other DNA
tgagagctccatagtgacacccaga

SEQ ID NO: 170 - DNA, 25 bp, synthetic construct
  source 1..25: mol_type = other DNA
ttccacatgtgagagctccatagtg

SEQ ID NO: 171 - DNA, 30 bp, synthetic construct
  source 1..30: mol_type = other DNA
aagaagaccttgcagcttccacatgtgaga

SEQ ID NO: 172 - DNA, 30 bp, synthetic construct
  source 1..30: mol_type = other DNA
gaagaagaccttgcagcttccacatgtgag

SEQ ID NO: 173 - DNA, 25 bp, synthetic construct
  source 1..25: mol_type = other DNA
aagaccttgcagcttccacatgtga

SEQ ID NO: 174 - DNA, 27 bp, synthetic construct
  source 1..27: mol_type = other DNA
aagaagaccttgcagcttccacatgtg

SEQ ID NO: 175 - DNA, 30 bp, synthetic construct
  source 1..30: mol_type = other DNA
ttgaagaagaccttgcagcttccacatgtg

SEQ ID NO: 176 - DNA, 27 bp, synthetic construct
  source 1..27: mol_type = other DNA
gaagaagaccttgcagcttccacatgt

SEQ ID NO: 177 - DNA, 30 bp, synthetic construct
  source 1..30: mol_type = other DNA
tttgaagaagaccttgcagcttccacatgt

SEQ ID NO: 178 - DNA, 27 bp, synthetic construct
  source 1..27: mol_type = other DNA
tgaagaagaccttgcagcttccacatg

SEQ ID NO: 179 - DNA, 25 bp, synthetic construct
  source 1..25: mol_type = other DNA
aagaagaccttgcagcttccacatg

SEQ ID NO: 180 - DNA, 27 bp, synthetic construct
  source 1..27: mol_type = other DNA
ttgaagaagaccttgcagcttccacat

SEQ ID NO: 181 - DNA, 25 bp, synthetic construct
  source 1..25: mol_type = other DNA
gaagaagaccttgcagcttccacat

SEQ ID NO: 182 - DNA, 27 bp, synthetic construct
  source 1..27: mol_type = other DNA
tttgaagaagaccttgcagcttccaca

SEQ ID NO: 183 - DNA, 25 bp, synthetic construct
  source 1..25: mol_type = other DNA
tgaagaagaccttgcagcttccaca

SEQ ID NO: 184 - DNA, 25 bp, synthetic construct
  source 1..25: mol_type = other DNA
ttgaagaagaccttgcagcttccac

SEQ ID NO: 185 - DNA, 25 bp, synthetic construct
  source 1..25: mol_type = other DNA
tttgaagaagaccttgcagcttcca

SEQ ID NO: 186 - DNA, 30 bp, synthetic construct
  source 1..30: mol_type = other DNA
caatcatttctgctggcgcacaggtacttc

SEQ ID NO: 187 - DNA, 30 bp, synthetic construct
  source 1..30: mol_type = other DNA
gcaatcatttctgctggcgcacaggtactt

SEQ ID NO: 188 - DNA, 27 bp, synthetic construct
  source 1..27: mol_type = other DNA
caatcatttctgctggcgcacaggtac

SEQ ID NO: 189 - DNA, 27 bp, synthetic construct
  source 1..27: mol_type = other DNA
gcaatcatttctgctggcgcacaggta

SEQ ID NO: 190 - DNA, 30 bp, synthetic construct
  source 1..30: mol_type = other DNA
agtgcaatcatttctgctggcgcacaggta

SEQ ID NO: 191 - DNA, 27 bp, synthetic construct
  source 1..27: mol_type = other DNA
tgcaatcatttctgctggcgcacaggt

SEQ ID NO: 192 - DNA, 25 bp, synthetic construct
  source 1..25: mol_type = other DNA
caatcatttctgctggcgcacaggt

SEQ ID NO: 193 - skipped

SEQ ID NO: 194 - DNA, 25 bp, synthetic construct
  source 1..25: mol_type = other DNA
gcaatcatttctgctggcgcacagg

SEQ ID NO: 195 - DNA, 27 bp, synthetic construct
  source 1..27: mol_type = other DNA
agtgcaatcatttctgctggcgcacag

SEQ ID NO: 196 - DNA, 30 bp, synthetic construct
  source 1..30: mol_type = other DNA
aatagtgcaatcatttctgctggcgcacag

SEQ ID NO: 197 - DNA, 25 bp, synthetic construct
  source 1..25: mol_type = other DNA
tgcaatcatttctgctggcgcacag

SEQ ID NO: 198 - DNA, 25 bp, synthetic construct
  source 1..25: mol_type = other DNA
gtgcaatcatttctgctggcgcaca

SEQ ID NO: 199 - DNA, 27 bp, synthetic construct
  source 1..27: mol_type = other DNA
atagtgcaatcatttctgctggcgcac

SEQ ID NO: 200 - DNA, 25 bp, synthetic construct
  source 1..25: mol_type = other DNA
agtgcaatcatttctgctggcgcac

SEQ ID NO: 201 - DNA, 27 bp, synthetic construct
  source 1..27: mol_type = other DNA
aatagtgcaatcatttctgctggcgca

SEQ ID NO: 202 - DNA, 25 bp, synthetic construct
  source 1..25: mol_type = other DNA
atagtgcaatcatttctgctggcgc

SEQ ID NO: 203 - DNA, 25 bp, synthetic construct
  source 1..25: mol_type = other DNA
aatagtgcaatcatttctgctggcg

SEQ ID NO: 204 - DNA, 27 bp, synthetic construct
  source 1..27: mol_type = other DNA
ggaatttatcaatagtgcaatcatttc

SEQ ID NO: 205 - DNA, 27 bp, synthetic construct
  source 1..27: mol_type = other DNA
cggaatttatcaatagtgcaatcattt

SEQ ID NO: 206 - DNA, 25 bp, synthetic construct
  source 1..25: mol_type = other DNA
ggaatttatcaatagtgcaatcatt

SEQ ID NO: 207 - DNA, 25 bp, synthetic construct
  source 1..25: mol_type = other DNA
cggaatttatcaatagtgcaatcat

SEQ ID NO: 208 - DNA, 30 bp, synthetic construct
  source 1..30: mol_type = other DNA
taacatttccgaagacgacaagatggacaa

SEQ ID NO: 209 - DNA, 30 bp, synthetic construct
  source 1..30: mol_type = other DNA
ataacatttccgaagacgacaagatggaca

SEQ ID NO: 210 - DNA, 30 bp, synthetic construct
  source 1..30: mol_type = other DNA
cataacatttccgaagacgacaagatggac

SEQ ID NO: 211 - DNA, 27 bp, synthetic construct
  source 1..27: mol_type = other DNA
taacatttccgaagacgacaagatgga

SEQ ID NO: 212 - DNA, 30 bp, synthetic construct
  source 1..30: mol_type = other DNA
tcataacatttccgaagacgacaagatgga

SEQ ID NO: 213 - DNA, 27 bp, synthetic construct
  source 1..27: mol_type = other DNA
ataacatttccgaagacgacaagatgg

SEQ ID NO: 214 - DNA, 30 bp, synthetic construct
  source 1..30: mol_type = other DNA
ttcataacatttccgaagacgacaagatgg

SEQ ID NO: 215 - DNA, 27 bp, synthetic construct
  source 1..27: mol_type = other DNA
cataacatttccgaagacgacaagatg

SEQ ID NO: 216 - DNA, 30 bp, synthetic construct
  source 1..30: mol_type = other DNA
cttcataacatttccgaagacgacaagatg

SEQ ID NO: 217 - DNA, 25 bp, synthetic construct
  source 1..25: mol_type = other DNA
taacatttccgaagacgacaagatg

SEQ ID NO: 218 - DNA, 27 bp, synthetic construct
  source 1..27: mol_type = other DNA
tcataacatttccgaagacgacaagat

SEQ ID NO: 219 - DNA, 25 bp, synthetic construct
  source 1..25: mol_type = other DNA
ataacatttccgaagacgacaagat

SEQ ID NO: 220 - DNA, 27 bp, synthetic construct
  source 1..27: mol_type = other DNA
ttcataacatttccgaagacgacaaga

SEQ ID NO: 221 - DNA, 25 bp, synthetic construct
  source 1..25: mol_type = other DNA
cataacatttccgaagacgacaaga

SEQ ID NO: 222 - DNA, 27 bp, synthetic construct
  source 1..27: mol_type = other DNA
cttcataacatttccgaagacgacaag

SEQ ID NO: 223 - DNA, 25 bp, synthetic construct
  source 1..25: mol_type = other DNA
tcataacatttccgaagacgacaag

SEQ ID NO: 224 - DNA, 25 bp, synthetic construct
  source 1..25: mol_type = other DNA
ttcataacatttccgaagacgacaa

SEQ ID NO: 225 - DNA, 25 bp, synthetic construct
  source 1..25: mol_type = other DNA
cttcataacatttccgaagacgaca

SEQ ID NO: 226 - DNA, 30 bp, synthetic construct
  source 1..30: mol_type = other DNA
gctcccagagtcatccctgcttcataacat

SEQ ID NO: 227 - DNA, 25 bp, synthetic construct
  source 1..25: mol_type = other DNA
attaccaagtttcttcagcttccgg

SEQ ID NO: 228 - DNA, 27 bp, synthetic construct
  source 1..27: mol_type = other DNA
cagattaccaagtttcttcagcttccg

SEQ ID NO: 229 - DNA, 25 bp, synthetic construct
  source 1..25: mol_type = other DNA
ttcaatgtgtgacactgtcagcttc

SEQ ID NO: 230 - DNA, 30 bp, synthetic construct
  source 1..30: mol_type = other DNA
atagccttcaatgtgtgacactgtcagctt

SEQ ID NO: 231 - DNA, 30 bp, synthetic construct
  source 1..30: mol_type = other DNA
catagccttcaatgtgtgacactgtcagct

SEQ ID NO: 232 - DNA, 27 bp, synthetic construct
  source 1..27: mol_type = other DNA
atagccttcaatgtgtgacactgtcag

SEQ ID NO: 233 - DNA, 25 bp, synthetic construct
  source 1..25: mol_type = other DNA
agccttcaatgtgtgacactgtcag

SEQ ID NO: 234 - DNA, 27 bp, synthetic construct
  source 1..27: mol_type = other DNA
catagccttcaatgtgtgacactgtca

SEQ ID NO: 235 - DNA, 25 bp, synthetic construct
  source 1..25: mol_type = other DNA
tagccttcaatgtgtgacactgtca

SEQ ID NO: 236 - DNA, 25 bp, synthetic construct
  source 1..25: mol_type = other DNA
atagccttcaatgtgtgacactgtc

SEQ ID NO: 237 - DNA, 25 bp, synthetic construct
  source 1..25: mol_type = other DNA
catagccttcaatgtgtgacactgt

SEQ ID NO: 238 - DNA, 30 bp, synthetic construct
  source 1..30: mol_type = other DNA
cattcagaaagatgggctgacattcatagc

SEQ ID NO: 239 - DNA, 30 bp, synthetic construct
  source 1..30: mol_type = other DNA
gacattcagaaagatgggctgacattcata

SEQ ID NO: 240 - DNA, 27 bp, synthetic construct
  source 1..27: mol_type = other DNA
cattcagaaagatgggctgacattcat

SEQ ID NO: 241 - DNA, 30 bp, synthetic construct
  source 1..30: mol_type = other DNA
ggacattcagaaagatgggctgacattcat

SEQ ID NO: 242 - DNA, 30 bp, synthetic construct
  source 1..30: mol_type = other DNA
aggacattcagaaagatgggctgacattca

SEQ ID NO: 243 - DNA, 27 bp, synthetic construct
  source 1..27: mol_type = other DNA
gacattcagaaagatgggctgacattc

SEQ ID NO: 244 - DNA, 25 bp, synthetic construct
  source 1..25: mol_type = other DNA
cattcagaaagatgggctgacattc

SEQ ID NO: 245 - DNA, 27 bp, synthetic construct
  source 1..27: mol_type = other DNA
ggacattcagaaagatgggctgacatt

SEQ ID NO: 246 - DNA, 27 bp, synthetic construct
  source 1..27: mol_type = other DNA
aggacattcagaaagatgggctgacat

SEQ ID NO: 247 - DNA, 25 bp, synthetic construct
  source 1..25: mol_type = other DNA
gacattcagaaagatgggctgacat

SEQ ID NO: 248 - DNA, 25 bp, synthetic construct
  source 1..25: mol_type = other DNA
ggacattcagaaagatgggctgaca

SEQ ID NO: 249 - DNA, 25 bp, synthetic construct
  source 1..25: mol_type = other DNA
aggacattcagaaagatgggctgac

SEQ ID NO: 250 - DNA, 27 bp, synthetic construct
  source 1..27: mol_type = other DNA
agcacacactacacctggctcaatggc

SEQ ID NO: 251 - DNA, 25 bp, synthetic construct
  source 1..25: mol_type = other DNA
agcacacactacacctggctcaatg

SEQ ID NO: 252 - DNA, 25 bp, synthetic construct
  source 1..25: mol_type = other DNA
ctggttgttgtcgtgtccagcacac

SEQ ID NO: 253 - DNA, 30 bp, synthetic construct
  source 1..30: mol_type = other DNA
ttcattgaggctagagagcaaggctgcaaa

SEQ ID NO: 254 - DNA, 30 bp, synthetic construct
  source 1..30: mol_type = other DNA
gttcattgaggctagagagcaaggctgcaa

SEQ ID NO: 255 - DNA, 30 bp, synthetic construct
  source 1..30: mol_type = other DNA
agttcattgaggctagagagcaaggctgca

SEQ ID NO: 256 - DNA, 25 bp, synthetic construct
  source 1..25: mol_type = other DNA
attgaggctagagagcaaggctgca

SEQ ID NO: 257 - DNA, 27 bp, synthetic construct
  source 1..27: mol_type = other DNA
ttcattgaggctagagagcaaggctgc

SEQ ID NO: 258 - DNA, 27 bp, synthetic construct
  source 1..27: mol_type = other DNA
gttcattgaggctagagagcaaggctg

SEQ ID NO: 259 - DNA, 27 bp, synthetic construct
  source 1..27: mol_type = other DNA
agttcattgaggctagagagcaaggct

SEQ ID NO: 260 - DNA, 25 bp, synthetic construct
  source 1..25: mol_type = other DNA
ttcattgaggctagagagcaaggct

SEQ ID NO: 261 - DNA, 25 bp, synthetic construct
  source 1..25: mol_type = other DNA
gttcattgaggctagagagcaaggc

SEQ ID NO: 262 - DNA, 25 bp, synthetic construct
  source 1..25: mol_type = other DNA
agttcattgaggctagagagcaagg

SEQ ID NO: 263 - DNA, 30 bp, synthetic construct
  source 1..30: mol_type = other DNA
gtacaagctgtctctctcccagttcattga

SEQ ID NO: 264 - DNA, 30 bp, synthetic construct
  source 1..30: mol_type = other DNA
tgtacaagctgtctctctcccagttcattg

SEQ ID NO: 265 - DNA, 27 bp, synthetic construct
  source 1..27: mol_type = other DNA
tacaagctgtctctctcccagttcatt

SEQ ID NO: 266 - DNA, 30 bp, synthetic construct
  source 1..30: mol_type = other DNA
gtgtacaagctgtctctctcccagttcatt

SEQ ID NO: 267 - DNA, 27 bp, synthetic construct
  source 1..27: mol_type = other DNA
gtacaagctgtctctctcccagttcat

SEQ ID NO: 268 - DNA, 30 bp, synthetic construct
  source 1..30: mol_type = other DNA
cgtgtacaagctgtctctctcccagttcat

SEQ ID NO: 269 - DNA, 27 bp, synthetic construct
  source 1..27: mol_type = other DNA
tgtacaagctgtctctctcccagttca

SEQ ID NO: 270 - DNA, 30 bp, synthetic construct
  source 1..30: mol_type = other DNA
acgtgtacaagctgtctctctcccagttca

SEQ ID NO: 271 - DNA, 25 bp, synthetic construct
  source 1..25: mol_type = other DNA
tacaagctgtctctctcccagttca

SEQ ID NO: 272 - DNA, 27 bp, synthetic construct
  source 1..27: mol_type = other DNA
gtgtacaagctgtctctctcccagttc

SEQ ID NO: 273 - DNA, 30 bp, synthetic construct
  source 1..30: mol_type = other DNA
cacgtgtacaagctgtctctctcccagttc

SEQ ID NO: 274 - DNA, 25 bp, synthetic construct
  source 1..25: mol_type = other DNA
gtacaagctgtctctctcccagttc

SEQ ID NO: 275 - DNA, 27 bp, synthetic construct
  source 1..27: mol_type = other DNA
cgtgtacaagctgtctctctcccagtt

SEQ ID NO: 276 - DNA, 25 bp, synthetic construct
  source 1..25: mol_type = other DNA
tgtacaagctgtctctctcccagtt

SEQ ID NO: 277 - DNA, 27 bp, synthetic construct
  source 1..27: mol_type = other DNA
acgtgtacaagctgtctctctcccagt

SEQ ID NO: 278 - DNA, 30 bp, synthetic construct
  source 1..30: mol_type = other DNA
accacgtgtacaagctgtctctctcccagt

SEQ ID NO: 279 - DNA, 25 bp, synthetic construct
  source 1..25: mol_type = other DNA
gtgtacaagctgtctctctcccagt

SEQ ID NO: 280 - DNA, 27 bp, synthetic construct
  source 1..27: mol_type = other DNA
cacgtgtacaagctgtctctctcccag

SEQ ID NO: 281 - DNA, 30 bp, synthetic construct
  source 1..30: mol_type = other DNA
gaccacgtgtacaagctgtctctctcccag

SEQ ID NO: 282 - DNA, 25 bp, synthetic construct
  source 1..25: mol_type = other DNA
cgtgtacaagctgtctctctcccag

SEQ ID NO: 283 - DNA, 30 bp, synthetic construct
  source 1..30: mol_type = other DNA
tgaccacgtgtacaagctgtctctctccca

SEQ ID NO: 284 - DNA, 25 bp, synthetic construct
  source 1..25: mol_type = other DNA
acgtgtacaagctgtctctctccca

SEQ ID NO: 285 - DNA, 27 bp, synthetic construct
  source 1..27: mol_type = other DNA
accacgtgtacaagctgtctctctccc

SEQ ID NO: 286 - DNA, 25 bp, synthetic construct
  source 1..25: mol_type = other DNA
cacgtgtacaagctgtctctctccc

SEQ ID NO: 287 - DNA, 27 bp, synthetic construct
  source 1..27: mol_type = other DNA
gaccacgtgtacaagctgtctctctcc

SEQ ID NO: 288 - DNA, 27 bp, synthetic construct
  source 1..27: mol_type = other DNA
tgaccacgtgtacaagctgtctctctc

SEQ ID NO: 289 - DNA, 25 bp, synthetic construct
  source 1..25: mol_type = other DNA
accacgtgtacaagctgtctctctc

SEQ ID NO: 290 - DNA, 25 bp, synthetic construct
  source 1..25: mol_type = other DNA
gaccacgtgtacaagctgtctctct

SEQ ID NO: 291 - DNA, 25 bp, synthetic construct
  source 1..25: mol_type = other DNA
tgaccacgtgtacaagctgtctctc

SEQ ID NO: 292 - DNA, 27 bp, synthetic construct
  source 1..27: mol_type = other DNA
cacgtgtaagttgcggaagccaggcaa

SEQ ID NO: 293 - DNA, 27 bp, synthetic construct
  source 1..27: mol_type = other DNA
tcgtccacgtgtaagttgcggaagcca

SEQ ID NO: 294 - DNA, 27 bp, synthetic construct
  source 1..27: mol_type = other DNA
acagccatctggtcgtccacgtgtaag

SEQ ID NO: 295 - DNA, 25 bp, synthetic construct
  source 1..25: mol_type = other DNA
acagccatctggtcgtccacgtgta

SEQ ID NO: 296 - DNA, 27 bp, synthetic construct
  source 1..27: mol_type = other DNA
aatgacagccatctggtcgtccacgtg

SEQ ID NO: 297 - DNA, 25 bp, synthetic construct
  source 1..25: mol_type = other DNA
aatgacagccatctggtcgtccacg

SEQ ID NO: 298 - DNA, 30 bp, synthetic construct
  source 1..30: mol_type = other DNA
agtactgaatgacagccatctggtcgtcca

SEQ ID NO: 299 - DNA, 27 bp, synthetic construct
  source 1..27: mol_type = other DNA
agtactgaatgacagccatctggtcgt

SEQ ID NO: 300 - DNA, 25 bp, synthetic construct
  source 1..25: mol_type = other DNA
gtactgaatgacagccatctggtcg

SEQ ID NO: 301 - skipped

SEQ ID NO: 302 - DNA, 27 bp, synthetic construct
  source 1..27: mol_type = other DNA
ccaggagtactgaatgacagccatctg

SEQ ID NO: 303 - DNA, 25 bp, synthetic construct
  source 1..25: mol_type = other DNA
aggagtactgaatgacagccatctg

SEQ ID NO: 304 - DNA, 25 bp, synthetic construct
  source 1..25: mol_type = other DNA
caggagtactgaatgacagccatct

SEQ ID NO: 305 - DNA, 25 bp, synthetic construct
  source 1..25: mol_type = other DNA
ccaggagtactgaatgacagccatc

SEQ ID NO: 306 - DNA, 25 bp, synthetic construct
  source 1..25: mol_type = other DNA
agttgacattggtgaaggatcgcca

SEQ ID NO: 307 - DNA, 30 bp, synthetic construct
  source 1..30: mol_type = other DNA
aactcttgagagaggtgcctcattcggaca

SEQ ID NO: 308 - DNA, 30 bp, synthetic construct
  source 1..30: mol_type = other DNA
aaactcttgagagaggtgcctcattcggac

SEQ ID NO: 309 - DNA, 30 bp, synthetic construct
  source 1..30: mol_type = other DNA
caaactcttgagagaggtgcctcattcgga

SEQ ID NO: 310 - DNA, 30 bp, synthetic construct
  source 1..30: mol_type = other DNA
ccaaactcttgagagaggtgcctcattcgg

SEQ ID NO: 311 - DNA, 27 bp, synthetic construct
  source 1..27: mol_type = other DNA
aaactcttgagagaggtgcctcattcg

SEQ ID NO: 312 - DNA, 27 bp, synthetic construct
  source 1..27: mol_type = other DNA
caaactcttgagagaggtgcctcattc

SEQ ID NO: 313 - DNA, 27 bp, synthetic construct
  source 1..27: mol_type = other DNA
ccaaactcttgagagaggtgcctcatt

SEQ ID NO: 314 - DNA, 25 bp, synthetic construct
  source 1..25: mol_type = other DNA
aaactcttgagagaggtgcctcatt

SEQ ID NO: 315 - DNA, 25 bp, synthetic construct
  source 1..25: mol_type = other DNA
caaactcttgagagaggtgcctcat

SEQ ID NO: 316 - DNA, 25 bp, synthetic construct
  source 1..25: mol_type = other DNA
ccaaactcttgagagaggtgcctca

SEQ ID NO: 317 - DNA, 27 bp, synthetic construct
  source 1..27: mol_type = other DNA
agtagcagtgctttcatgcacaggaat

SEQ ID NO: 318 - DNA, 30 bp, synthetic construct
  source 1..30: mol_type = other DNA
aatgctgaagagtagcagtgctttcatgca

SEQ ID NO: 319 - DNA, 27 bp, synthetic construct
  source 1..27: mol_type = other DNA
aatgctgaagagtagcagtgctttcat

SEQ ID NO: 320 - DNA, 30 bp, synthetic construct
  source 1..30: mol_type = other DNA
aataatgctgaagagtagcagtgctttcat

SEQ ID NO: 321 - DNA, 30 bp, synthetic construct
  source 1..30: mol_type = other DNA
gaataatgctgaagagtagcagtgctttca

SEQ ID NO: 322 - DNA, 30 bp, synthetic construct
  source 1..30: mol_type = other DNA
ggaataatgctgaagagtagcagtgctttc

SEQ ID NO: 323 - DNA, 25 bp, synthetic construct
  source 1..25: mol_type = other DNA
aatgctgaagagtagcagtgctttc

SEQ ID NO: 324 - DNA, 27 bp, synthetic construct
  source 1..27: mol_type = other DNA
aataatgctgaagagtagcagtgcttt

SEQ ID NO: 325 - DNA, 27 bp, synthetic construct
  source 1..27: mol_type = other DNA
gaataatgctgaagagtagcagtgctt

SEQ ID NO: 326 - DNA, 27 bp, synthetic construct
  source 1..27: mol_type = other DNA
ggaataatgctgaagagtagcagtgct

SEQ ID NO: 327 - DNA, 25 bp, synthetic construct
  source 1..25: mol_type = other DNA
aataatgctgaagagtagcagtgct

SEQ ID NO: 328 - DNA, 25 bp, synthetic construct
  source 1..25: mol_type = other DNA
gaataatgctgaagagtagcagtgc

SEQ ID NO: 329 - DNA, 25 bp, synthetic construct
  source 1..25: mol_type = other DNA
ggaataatgctgaagagtagcagtg

SEQ ID NO: 330 - DNA, 30 bp, synthetic construct
  source 1..30: mol_type = other DNA
tgcaatgatacgatcgagttccttgatgta

SEQ ID NO: 331 - DNA, 27 bp, synthetic construct
  source 1..27: mol_type = other DNA
tgcaatgatacgatcgagttccttgat

SEQ ID NO: 332 - DNA, 30 bp, synthetic construct
  source 1..30: mol_type = other DNA
tgcatgcaatgatacgatcgagttccttga

SEQ ID NO: 333 - DNA, 30 bp, synthetic construct
  source 1..30: mol_type = other DNA
ttgcatgcaatgatacgatcgagttccttg

SEQ ID NO: 334 - DNA, 25 bp, synthetic construct
  source 1..25: mol_type = other DNA
tgcaatgatacgatcgagttccttg

SEQ ID NO: 335 - DNA, 30 bp, synthetic construct
  source 1..30: mol_type = other DNA
tttgcatgcaatgatacgatcgagttcctt

SEQ ID NO: 336 - DNA, 27 bp, synthetic construct
  source 1..27: mol_type = other DNA
tgcatgcaatgatacgatcgagttcct

SEQ ID NO: 337 - DNA, 27 bp, synthetic construct
  source 1..27: mol_type = other DNA
ttgcatgcaatgatacgatcgagttcc

SEQ ID NO: 338 - DNA, 27 bp, synthetic construct
  source 1..27: mol_type = other DNA
tttgcatgcaatgatacgatcgagttc

SEQ ID NO: 339 - DNA, 25 bp, synthetic construct
  source 1..25: mol_type = other DNA
tgcatgcaatgatacgatcgagttc

SEQ ID NO: 340 - DNA, 25 bp, synthetic construct
  source 1..25: mol_type = other DNA
ttgcatgcaatgatacgatcgagtt

SEQ ID NO: 341 - DNA, 25 bp, synthetic construct
  source 1..25: mol_type = other DNA
tttgcatgcaatgatacgatcgagt

SEQ ID NO: 342 - DNA, 30 bp, synthetic construct
  source 1..30: mol_type = other DNA
aagtgaactgatgcagctctctcgcaatag

SEQ ID NO: 343 - DNA, 30 bp, synthetic construct
  source 1..30: mol_type = other DNA
aaagtgaactgatgcagctctctcgcaata

SEQ ID NO: 344 - DNA, 27 bp, synthetic construct
  source 1..27: mol_type = other DNA
aagtgaactgatgcagctctctcgcaa

SEQ ID NO: 345 - DNA, 27 bp, synthetic construct
  source 1..27: mol_type = other DNA
aaagtgaactgatgcagctctctcgca

SEQ ID NO: 346 - DNA, 25 bp, synthetic construct
  source 1..25: mol_type = other DNA
aaagtgaactgatgcagctctctcg

SEQ ID NO: 347 - DNA, 30 bp, synthetic construct
  source 1..30: mol_type = other DNA
atttccggaaagtccacgctcaccatgtgt

SEQ ID NO: 348 - DNA, 27 bp, synthetic construct
  source 1..27: mol_type = other DNA
ttccggaaagtccacgctcaccatgtg

SEQ ID NO: 349 - DNA, 30 bp, synthetic construct
  source 1..30: mol_type = other DNA
catttccggaaagtccacgctcaccatgtg

SEQ ID NO: 350 - DNA, 27 bp, synthetic construct
  source 1..27: mol_type = other DNA
tttccggaaagtccacgctcaccatgt

SEQ ID NO: 351 - DNA, 30 bp, synthetic construct
  source 1..30: mol_type = other DNA
tcatttccggaaagtccacgctcaccatgt

SEQ ID NO: 352 - DNA, 27 bp, synthetic construct
  source 1..27: mol_type = other DNA
atttccggaaagtccacgctcaccatg

SEQ ID NO: 353 - DNA, 30 bp, synthetic construct
  source 1..30: mol_type = other DNA
atcatttccggaaagtccacgctcaccatg

SEQ ID NO: 354 - DNA, 25 bp, synthetic construct
  source 1..25: mol_type = other DNA
ttccggaaagtccacgctcaccatg

SEQ ID NO: 355 - DNA, 27 bp, synthetic construct
  source 1..27: mol_type = other DNA
catttccggaaagtccacgctcaccat

SEQ ID NO: 356 - DNA, 30 bp, synthetic construct
  source 1..30: mol_type = other DNA
catcatttccggaaagtccacgctcaccat

SEQ ID NO: 357 - DNA, 25 bp, synthetic construct
  source 1..25: mol_type = other DNA
tttccggaaagtccacgctcaccat

SEQ ID NO: 358 - DNA, 27 bp, synthetic construct
  source 1..27: mol_type = other DNA
tcatttccggaaagtccacgctcacca

SEQ ID NO: 359 - DNA, 30 bp, synthetic construct
  source 1..30: mol_type = other DNA
ccatcatttccggaaagtccacgctcacca

SEQ ID NO: 360 - DNA, 25 bp, synthetic construct
  source 1..25: mol_type = other DNA
atttccggaaagtccacgctcacca

SEQ ID NO: 361 - DNA, 27 bp, synthetic construct
  source 1..27: mol_type = other DNA
atcatttccggaaagtccacgctcacc

SEQ ID NO: 362 - DNA, 25 bp, synthetic construct
  source 1..25: mol_type = other DNA
catttccggaaagtccacgctcacc

SEQ ID NO: 363 - DNA, 27 bp, synthetic construct
  source 1..27: mol_type = other DNA
catcatttccggaaagtccacgctcac

SEQ ID NO: 364 - DNA, 25 bp, synthetic construct
  source 1..25: mol_type = other DNA
tcatttccggaaagtccacgctcac

SEQ ID NO: 365 - DNA, 27 bp, synthetic construct
  source 1..27: mol_type = other DNA
ccatcatttccggaaagtccacgctca

SEQ ID NO: 366 - DNA, 25 bp, synthetic construct
  source 1..25: mol_type = other DNA
atcatttccggaaagtccacgctca

SEQ ID NO: 367 - DNA, 25 bp, synthetic construct
  source 1..25: mol_type = other DNA
catcatttccggaaagtccacgctc

SEQ ID NO: 368 - DNA, 25 bp, synthetic construct
  source 1..25: mol_type = other DNA
ccatcatttccggaaagtccacgct

SEQ ID NO: 369 - DNA, 30 bp, synthetic construct
  source 1..30: mol_type = other DNA
cagaaaggatcttgggcacttgcacagaga

SEQ ID NO: 370 - DNA, 30 bp, synthetic construct
  source 1..30: mol_type = other DNA
ccagaaaggatcttgggcacttgcacagag

SEQ ID NO: 371 - DNA, 30 bp, synthetic construct
  source 1..30: mol_type = other DNA
cccagaaaggatcttgggcacttgcacaga

SEQ ID NO: 372 - DNA, 27 bp, synthetic construct
  source 1..27: mol_type = other DNA
cagaaaggatcttgggcacttgcacag

SEQ ID NO: 373 - DNA, 27 bp, synthetic construct
  source 1..27: mol_type = other DNA
ccagaaaggatcttgggcacttgcaca

SEQ ID NO: 374 - DNA, 27 bp, synthetic construct
  source 1..27: mol_type = other DNA
cccagaaaggatcttgggcacttgcac

SEQ ID NO: 375 - DNA, 25 bp, synthetic construct
  source 1..25: mol_type = other DNA
cagaaaggatcttgggcacttgcac

SEQ ID NO: 376 - DNA, 25 bp, synthetic construct
  source 1..25: mol_type = other DNA
cccagaaaggatcttgggcacttgc

SEQ ID NO: 377 - DNA, 30 bp, synthetic construct
  source 1..30: mol_type = other DNA
aaatagatgggcttgactttcccagaaagg

SEQ ID NO: 378 - DNA, 27 bp, synthetic construct
  source 1..27: mol_type = other DNA
aaatagatgggcttgactttcccagaa

SEQ ID NO: 379 - protein, 20 aa, synthetic construct
KRKGDEVDGVDEVAKKKSKK

SEQ ID NO: 380 - DNA, 21 bp, synthetic construct
  source 1..21: mol_type = other DNA
gacgaccagatggctgtcatt

SEQ ID NO: 381 - DNA, 19 bp, synthetic construct
  source 1..19: mol_type = other DNA
gggcgaagtagagcatcct

SEQ ID NO: 382 - DNA, 19 bp, synthetic construct
  source 1..19: mol_type = other DNA
ccagggaccatgttttgcc

SEQ ID NO: 383 - DNA, 21 bp, synthetic construct
  source 1..21: mol_type = other DNA
cgaagacgacaagatggacaa

SEQ ID NO: 384 - DNA, 20 bp, synthetic construct
  source 1..20: mol_type = other DNA
ccatggggaaggtgaaggtc

SEQ ID NO: 385 - DNA, 21 bp, synthetic construct
  source 1..21: mol_type = other DNA
gaaggggtcattgatggcaac

SEQ ID NO: 386 - protein, 17 aa, synthetic construct
RKCLQAGMNLEARKTKK

SEQ ID NO: 387 - DNA, 4780 bp, synthetic construct
  source 1..4780: mol_type = other DNA
cctgcaggcagctgcgcgctcgctcgctcactgaggccgcccgggcgtcgggcgacctttggtcgcccggcctcagtgagcgagcgagcgcgcagagagggagtggccaactccatcactaggggttcctgcggcctctagactcgaggcgttgacattgattattgactagttattaatagtaatcaattacggggtcattagttcatagcccatatatggagttccgcgttacataacttacggtaaatggcccgcctggctgaccgcccaacgacccccgcccattgacgtcaataatgacgtatgttcccatagtaacgccaatagggactttccattgacgtcaatgggtggagtatttacggtaaactgcccacttggcagtacatcaagtgtatcatatgccaagtacgccccctattgacgtcaatgacggtaaatggcccgcctggcattatgcccagtacatgaccttatgggactttcctacttggcagtacatctacgtattagtcatcgctattaccatggtgatgcggttttggcagtacatcaatgggcgtggatagcggtttgactcacggggatttccaagtctccaccccattgacgtcaatgggagtttgttttggcaccaaaatcaacgggactttccaaaatgtcgtaacaactccgccccattgacgcaaatgggcggtaggcgtgtacggtgggaggtctatataagcagagctctctggctaactaccggtgccaccatggtgagcaagggcgaggagctgttcaccggggtggtgcccatcctggtcgagctggacggcgacgtaaacggccacaagttcagcgtgtccggcgagggcgagggcgatgccacctacggcaagctgaccctgaagttcatctgcaccaccggcaagctgcccgtgccctggcccaccctcgtgaccaccctgacctacggcgtgcagtgcttcagccgctaccccgaccacatgaagcagcacgacttcttcaagtccgccatgcccgaaggctacgtccaggagcgcaccatcttcttcaaggacgacggcaactacaagacccgcgccgaggtgaagttcgagggcgacaccctggtgaaccgcatcgagctgaagggcatcgacttcaaggaggacggcaacatcctggggcacaagctggagtacaactacaacagccacaacgtctatatcatggccgacaagcagaagaacggcatcaaggtgaacttcaagatccgccacaacatcgaggacggcagcgtgcagctcgccgaccactaccagcagaacacccccatcggcgacggccccgtgctgctgcccgacaaccactacctgagcacccagtccgccctgagcaaagaccccaacgagaagcgcgatcacatggtcctgctggagttcgtgaccgccgccgggatcactctcggcatggacgagctgtacaagtaaagcggccgaattcctagagctcgctgatcagcctcgactgtgccttctagttgccagccatctgttgtttgcccctcccccgtgccttccttgaccctggaaggtgccactcccactgtcctttcctaataaaatgaggaaattgcatcgcattgtctgagtaggtgtcattctattctggggggtggggtggggcaggacagcaagggggaggattgggaagagaatagcaggcatgctggggaggtaccgagggcctatttcccatgattccttcatatttgcatatacgatacaaggctgttagagagataattggaattaatttgactgtaaacacaaagatattagtacaaaatacgtgacgtagaaagtaataatttcttgggtagtttgcagttttaaaattatgttttaaaatggactatcatatgcttaccgtaacttgaaagtatttcgatttcttggctttatatatcttgtggaaaggacgaaacaccggttcacttttgacctgctaatctcgagattagcaggtcaaaagtgaacttttttggccgcaggaacccctagtgatggagttggccactccctctctgcgcgctcgctcgctcactgaggccgggcgaccaaaggtcgcccgacgcccgggctttgcccgggcggcctcagtgagcgagcgagcgcgcagctgcctgcaggggcgcctgatgcggtattttctccttacgcatctgtgcggtatttcacaccgcatacgtcaaagcaaccatagtacgcgccctgtagcggcgcattaagcgcggcgggtgtggtggttacgcgcagcgtgaccgctacacttgccagcgccctagcgcccgctcctttcgctttcttcccttcctttctcgccacgttcgccggctttccccgtcaagctctaaatcgggggctccctttagggttccgatttagtgctttacggcacctcgaccccaaaaaacttgatttgggtgatggttcacgtagtgggccatcgccctgatagacggtttttcgccctttgacgttggagtccacgttctttaatagtggactcttgttccaaactggaacaacactcaaccctatctcgggctattcttttgatttataagggattttgccgatttcggcctattggttaaaaaatgagctgatttaacaaaaatttaacgcgaattttaacaaaatattaacgtttacaattttatggtgcactctcagtacaatctgctctgatgccgcatagttaagccagccccgacacccgccaacacccgctgacgcgccctgacgggcttgtctgctcccggcatccgcttacagacaagctgtgaccgtctccgggagctgcatgtgtcagaggttttcaccgtcatcaccgaaacgcgcgagacgaaagggcctcgtgatacgcctatttttataggttaatgtcatgataataatggtttcttagacgtcaggtggcacttttcggggaaatgtgcgcggaacccctatttgtttatttttctaaatacattcaaatatgtatccgctcatgagacaataaccctgataaatgcttcaataatattgaaaaaggaagagtatgagtattcaacatttccgtgtcgcccttattcccttttttgcggcattttgccttcctgtttttgctcacccagaaacgctggtgaaagtaaaagatgctgaagatcagttgggtgcacgagtgggttacatcgaactggatctcaacagcggtaagatccttgagagttttcgccccgaagaacgttttccaatgatgagcacttttaaagttctgctatgtggcgcggtattatcccgtattgacgccgggcaagagcaactcggtcgccgcatacactattctcagaatgacttggttgagtactcaccagtcacagaaaagcatcttacggatggcatgacagtaagagaattatgcagtgctgccataaccatgagtgataacactgcggccaacttacttctgacaacgatcggaggaccgaaggagctaaccgcttttttgcacaacatgggggatcatgtaactcgccttgatcgttgggaaccggagctgaatgaagccataccaaacgacgagcgtgacaccacgatgcctgtagcaatggcaacaacgttgcgcaaactattaactggcgaactacttactctagcttcccggcaacaattaatagactggatggaggcggataaagttgcaggaccacttctgcgctcggcccttccggctggctggtttattgctgataaatctggagccggtgagcgtggaagccgcggtatcattgcagcactggggccagatggtaagccctcccgtatcgtagttatctacacgacggggagtcaggcaactatggatgaacgaaatagacagatcgctgagataggtgcctcactgattaagcattggtaactgtcagaccaagtttactcatatatactttagattgatttaaaacttcatttttaatttaaaaggatctaggtgaagatcctttttgataatctcatgaccaaaatcccttaacgtgagttttcgttccactgagcgtcagaccccgtagaaaagatcaaaggatcttcttgagatcctttttttctgcgcgtaatctgctgcttgcaaacaaaaaaaccaccgctaccagcggtggtttgtttgccggatcaagagctaccaactctttttccgaaggtaactggcttcagcagagcgcagataccaaatactgtccttctagtgtagccgtagttaggccaccacttcaagaactctgtagcaccgcctacatacctcgctctgctaatcctgttaccagtggctgctgccagtggcgataagtcgtgtcttaccgggttggactcaagacgatagttaccggataaggcgcagcggtcgggctgaacggggggttcgtgcacacagcccagcttggagcgaacgacctacaccgaactgagatacctacagcgtgagctatgagaaagcgccacgcttcccgaagggagaaaggcggacaggtatccggtaagcggcagggtcggaacaggagagcgcacgagggagcttccagggggaaacgcctggtatctttatagtcctgtcgggtttcgccacctctgacttgagcgtcgatttttgtgatgctcgtcaggggggcggagcctatggaaaaacgccagcaacgcggcctttttacggttcctggccttttgctggccttttgctcacatgt

SEQ ID NO: 388 - DNA, 4776 bp, synthetic construct
  source 1..4776: mol_type = other DNA
cctgcaggcagctgcgcgctcgctcgctcactgaggccgcccgggcgtcgggcgacctttggtcgcccggcctcagtgagcgagcgagcgcgcagagagggagtggccaactccatcactaggggttcctgcggcctctagactcgaggcgttgacattgattattgactagttattaatagtaatcaattacggggtcattagttcatagcccatatatggagttccgcgttacataacttacggtaaatggcccgcctggctgaccgcccaacgacccccgcccattgacgtcaataatgacgtatgttcccatagtaacgccaatagggactttccattgacgtcaatgggtggagtatttacggtaaactgcccacttggcagtacatcaagtgtatcatatgccaagtacgccccctattgacgtcaatgacggtaaatggcccgcctggcattatgcccagtacatgaccttatgggactttcctacttggcagtacatctacgtattagtcatcgctattaccatggtgatgcggttttggcagtacatcaatgggcgtggatagcggtttgactcacggggatttccaagtctccaccccattgacgtcaatgggagtttgttttggcaccaaaatcaacgggactttccaaaatgtcgtaacaactccgccccattgacgcaaatgggcggtaggcgtgtacggtgggaggtctatataagcagagctctctggctaactaccggtgccaccatggtgagcaagggcgaggagctgttcaccggggtggtgcccatcctggtcgagctggacggcgacgtaaacggccacaagttcagcgtgtccggcgagggcgagggcgatgccacctacggcaagctgaccctgaagttcatctgcaccaccggcaagctgcccgtgccctggcccaccctcgtgaccaccctgacctacggcgtgcagtgcttcagccgctaccccgaccacatgaagcagcacgacttcttcaagtccgccatgcccgaaggctacgtccaggagcgcaccatcttcttcaaggacgacggcaactacaagacccgcgccgaggtgaagttcgagggcgacaccctggtgaaccgcatcgagctgaagggcatcgacttcaaggaggacggcaacatcctggggcacaagctggagtacaactacaacagccacaacgtctatatcatggccgacaagcagaagaacggcatcaaggtgaacttcaagatccgccacaacatcgaggacggcagcgtgcagctcgccgaccactaccagcagaacacccccatcggcgacggccccgtgctgctgcccgacaaccactacctgagcacccagtccgccctgagcaaagaccccaacgagaagcgcgatcacatggtcctgctggagttcgtgaccgccgccgggatcactctcggcatggacgagctgtacaagtaaagcggccgaattcctagagctcgctgatcagcctcgactgtgccttctagttgccagccatctgttgtttgcccctcccccgtgccttccttgaccctggaaggtgccactcccactgtcctttcctaataaaatgaggaaattgcatcgcattgtctgagtaggtgtcattctattctggggggtggggtggggcaggacagcaagggggaggattgggaagagaatagcaggcatgctggggaggtaccgagggcctatttcccatgattccttcatatttgcatatacgatacaaggctgttagagagataattggaattaatttgactgtaaacacaaagatattagtacaaaatacgtgacgtagaaagtaataatttcttgggtagtttgcagttttaaaattatgttttaaaatggactatcatatgcttaccgtaacttgaaagtatttcgatttcttggctttatatatcttgtggaaaggacgaaacaccggacctaccgaggagctttcctcgaggaaagctcctcggtaggtcttttttggccgcaggaacccctagtgatggagttggccactccctctctgcgcgctcgctcgctcactgaggccgggcgaccaaaggtcgcccgacgcccgggctttgcccgggcggcctcagtgagcgagcgagcgcgcagctgcctgcaggggcgcctgatgcggtattttctccttacgcatctgtgcggtatttcacaccgcatacgtcaaagcaaccatagtacgcgccctgtagcggcgcattaagcgcggcgggtgtggtggttacgcgcagcgtgaccgctacacttgccagcgccctagcgcccgctcctttcgctttcttcccttcctttctcgccacgttcgccggctttccccgtcaagctctaaatcgggggctccctttagggttccgatttagtgctttacggcacctcgaccccaaaaaacttgatttgggtgatggttcacgtagtgggccatcgccctgatagacggtttttcgccctttgacgttggagtccacgttctttaatagtggactcttgttccaaactggaacaacactcaaccctatctcgggctattcttttgatttataagggattttgccgatttcggcctattggttaaaaaatgagctgatttaacaaaaatttaacgcgaattttaacaaaatattaacgtttacaattttatggtgcactctcagtacaatctgctctgatgccgcatagttaagccagccccgacacccgccaacacccgctgacgcgccctgacgggcttgtctgctcccggcatccgcttacagacaagctgtgaccgtctccgggagctgcatgtgtcagaggttttcaccgtcatcaccgaaacgcgcgagacgaaagggcctcgtgatacgcctatttttataggttaatgtcatgataataatggtttcttagacgtcaggtggcacttttcggggaaatgtgcgcggaacccctatttgtttatttttctaaatacattcaaatatgtatccgctcatgagacaataaccctgataaatgcttcaataatattgaaaaaggaagagtatgagtattcaacatttccgtgtcgcccttattcccttttttgcggcattttgccttcctgtttttgctcacccagaaacgctggtgaaagtaaaagatgctgaagatcagttgggtgcacgagtgggttacatcgaactggatctcaacagcggtaagatccttgagagttttcgccccgaagaacgttttccaatgatgagcacttttaaagttctgctatgtggcgcggtattatcccgtattgacgccgggcaagagcaactcggtcgccgcatacactattctcagaatgacttggttgagtactcaccagtcacagaaaagcatcttacggatggcatgacagtaagagaattatgcagtgctgccataaccatgagtgataacactgcggccaacttacttctgacaacgatcggaggaccgaaggagctaaccgcttttttgcacaacatgggggatcatgtaactcgccttgatcgttgggaaccggagctgaatgaagccataccaaacgacgagcgtgacaccacgatgcctgtagcaatggcaacaacgttgcgcaaactattaactggcgaactacttactctagcttcccggcaacaattaatagactggatggaggcggataaagttgcaggaccacttctgcgctcggcccttccggctggctggtttattgctgataaatctggagccggtgagcgtggaagccgcggtatcattgcagcactggggccagatggtaagccctcccgtatcgtagttatctacacgacggggagtcaggcaactatggatgaacgaaatagacagatcgctgagataggtgcctcactgattaagcattggtaactgtcagaccaagtttactcatatatactttagattgatttaaaacttcatttttaatttaaaaggatctaggtgaagatcctttttgataatctcatgaccaaaatcccttaacgtgagttttcgttccactgagcgtcagaccccgtagaaaagatcaaaggatcttcttgagatcctttttttctgcgcgtaatctgctgcttgcaaacaaaaaaaccaccgctaccagcggtggtttgtttgccggatcaagagctaccaactctttttccgaaggtaactggcttcagcagagcgcagataccaaatactgtccttctagtgtagccgtagttaggccaccacttcaagaactctgtagcaccgcctacatacctcgctctgctaatcctgttaccagtggctgctgccagtggcgataagtcgtgtcttaccgggttggactcaagacgatagttaccggataaggcgcagcggtcgggctgaacggggggttcgtgcacacagcccagcttggagcgaacgacctacaccgaactgagatacctacagcgtgagctatgagaaagcgccacgcttcccgaagggagaaaggcggacaggtatccggtaagcggcagggtcggaacaggagagcgcacgagggagcttccagggggaaacgcctggtatctttatagtcctgtcgggtttcgccacctctgacttgagcgtcgatttttgtgatgctcgtcaggggggcggagcctatggaaaaacgccagcaacgcggcctttttacggttcctggccttttgctggccttttgctcacatgt

SEQ ID NO: 389 - protein, 10 aa, synthetic construct
RKLKKKIKKL

SEQ ID NO: 390 - DNA, 21 bp, synthetic construct
  source 1..21: mol_type = other DNA
gttcacttttgacctgctaat

SEQ ID NO: 391 - DNA, 19 bp, synthetic construct
  source 1..19: mol_type = other DNA
gacctaccgaggagctttc

SEQ ID NO: 392 - protein, 10 aa, synthetic construct
REKKKFLKRR

SEQ ID NO: 393 - DNA, 30 bp, synthetic construct
  source 1..30: mol_type = other DNA
tgccgttcttctgcttgtcggccatgatat

SEQ ID NO: 394 - DNA, 10667 bp, Homo sapiens
  source 1..10667: mol_type = other DNA
agcgccccctccgagatcccggggagccagcttgctgggagagcgggacggtccggagcaagcccagaggcagaggaggcgacagagggaaaaagggccgagctagccgctccagtgctgtacaggagccgaagggacgcaccacgccagccccagcccggctccagcgacagccaacgcctcttgcagcgcggcggcttcgaagccgccgcccggagctgccctttcctcttcggtgaagtttttaaaagctgctaaagactcggaggaagcaaggaaagtgcctggtaggactgacggctgcctttgtcctcctcctctccaccccgcctccccccaccctgccttccccccctcccccgtcttctctcccgcagctgcctcagtcggctactctcagccaacccccctcaccacccttctccccacccgcccccccgcccccgtcggcccagcgctgccagcccgagtttgcagagaggtaactccctttggctgcgagcgggcgagctagctgcacattgcaaagaaggctcttaggagccaggcgactggggagcggcttcagcactgcagccacgacccgcctggttaggctgcacgcggagagaaccctctgttttcccccactctctctccacctcctcctgccttccccaccccgagtgcggagccagagatcaaaagatgaaaaggcagtcaggtcttcagtagccaaaaaacaaaacaaacaaaaacaaaaaagccgaaataaaagaaaaagataataactcagttcttatttgcacctacttcagtggacactgaatttggaaggtggaggattttgtttttttcttttaagatctgggcatcttttgaatctacccttcaagtattaagagacagactgtgagcctagcagggcagatcttgtccaccgtgtgtcttcttctgcacgagactttgaggctgtcagagcgctttttgcgtggttgctcccgcaagtttccttctctggagcttcccgcaggtgggcagctagctgcagcgactaccgcatcatcacagcctgttgaactcttctgagcaagagaaggggaggcggggtaagggaagtaggtggaagattcagccaagctcaaggatggaagtgcagttagggctgggaagggtctaccctcggccgccgtccaagacctaccgaggagctttccagaatctgttccagagcgtgcgcgaagtgatccagaacccgggccccaggcacccagaggccgcgagcgcagcacctcccggcgccagtttgctgctgctgcagcagcagcagcagcagcagcagcagcagcagcagcagcagcagcagcagcagcagcagcagcagcaagagactagccccaggcagcagcagcagcagcagggtgaggatggttctccccaagcccatcgtagaggccccacaggctacctggtcctggatgaggaacagcaaccttcacagccgcagtcggccctggagtgccaccccgagagaggttgcgtcccagagcctggagccgccgtggccgccagcaaggggctgccgcagcagctgccagcacctccggacgaggatgactcagctgccccatccacgttgtccctgctgggccccactttccccggcttaagcagctgctccgctgaccttaaagacatcctgagcgaggccagcaccatgcaactccttcagcaacagcagcaggaagcagtatccgaaggcagcagcagcgggagagcgagggaggcctcgggggctcccacttcctccaaggacaattacttagggggcacttcgaccatttctgacaacgccaaggagttgtgtaaggcagtgtcggtgtccatgggcctgggtgtggaggcgttggagcatctgagtccaggggaacagcttcggggggattgcatgtacgccccacttttgggagttccacccgctgtgcgtcccactccttgtgccccattggccgaatgcaaaggttctctgctagacgacagcgcaggcaagagcactgaagatactgctgagtattcccctttcaagggaggttacaccaaagggctagaaggcgagagcctaggctgctctggcagcgctgcagcagggagctccgggacacttgaactgccgtctaccctgtctctctacaagtccggagcactggacgaggcagctgcgtaccagagtcgcgactactacaactttccactggctctggccggaccgccgccccctccgccgcctccccatccccacgctcgcatcaagctggagaacccgctggactacggcagcgcctgggcggctgcggcggcgcagtgccgctatggggacctggcgagcctgcatggcgcgggtgcagcgggacccggttctgggtcaccctcagccgccgcttcctcatcctggcacactctcttcacagccgaagaaggccagttgtatggaccgtgtggtggtggtgggggtggtggcggcggcggcggcggcggcggcggcggcggcggcggcggcggcggcggcgaggcgggagctgtagccccctacggctacactcggccccctcaggggctggcgggccaggaaagcgacttcaccgcacctgatgtgtggtaccctggcggcatggtgagcagagtgccctatcccagtcccacttgtgtcaaaagcgaaatgggcccctggatggatagctactccggaccttacggggacatgcgtttggagactgccagggaccatgttttgcccattgactattactttccaccccagaagacctgcctgatctgtggagatgaagcttctgggtgtcactatggagctctcacatgtggaagctgcaaggtcttcttcaaaagagccgctgaagggaaacagaagtacctgtgcgccagcagaaatgattgcactattgataaattccgaaggaaaaattgtccatcttgtcgtcttcggaaatgttatgaagcagggatgactctgggagcccggaagctgaagaaacttggtaatctgaaactacaggaggaaggagaggcttccagcaccaccagccccactgaggagacaacccagaagctgacagtgtcacacattgaaggctatgaatgtcagcccatctttctgaatgtcctggaagccattgagccaggtgtagtgtgtgctggacacgacaacaaccagcccgactcctttgcagccttgctctctagcctcaatgaactgggagagagacagcttgtacacgtggtcaagtgggccaaggccttgcctggcttccgcaacttacacgtggacgaccagatggctgtcattcagtactcctggatggggctcatggtgtttgccatgggctggcgatccttcaccaatgtcaactccaggatgctctacttcgcccctgatctggttttcaatgagtaccgcatgcacaagtcccggatgtacagccagtgtgtccgaatgaggcacctctctcaagagtttggatggctccaaatcaccccccaggaattcctgtgcatgaaagcactgctactcttcagcattattccagtggatgggctgaaaaatcaaaaattctttgatgaacttcgaatgaactacatcaaggaactcgatcgtatcattgcatgcaaaagaaaaaatcccacatcctgctcaagacgcttctaccagctcaccaagctcctggactccgtgcagcctattgcgagagagctgcatcagttcacttttgacctgctaatcaagtcacacatggtgagcgtggactttccggaaatgatggcagagatcatctctgtgcaagtgcccaagatcctttctgggaaagtcaagcccatctatttccacacccagtgaagcattggaaaccctatttccccaccccagctcatgccccctttcagatgtcttctgcctgttataactctgcactactcctctgcagtgccttggggaatttcctctattgatgtacagtctgtcatgaacatgttcctgaattctatttgctgggctttttttttctctttctctcctttctttttcttcttccctccctatctaaccctcccatggcaccttcagactttgcttcccattgtggctcctatctgtgttttgaatggtgttgtatgcctttaaatctgtgatgatcctcatatggcccagtgtcaagttgtgcttgtttacagcactactctgtgccagccacacaaacgtttacttatcttatgccacgggaagtttagagagctaagattatctggggaaatcaaaacaaaaacaagcaaacaaaaaaaaaaagcaaaaacaaaacaaaaaataagccaaaaaaccttgctagtgttttttcctcaaaaataaataaataaataaataaatacgtacatacatacacacatacatacaaacatatagaaatccccaaagaggccaatagtgacgagaaggtgaaaattgcaggcccatggggagttactgattttttcatctcctccctccacgggagactttattttctgccaatggctattgccattagagggcagagtgaccccagagctgagttgggcaggggggtggacagagaggagaggacaaggagggcaatggagcatcagtacctgcccacagccttggtccctgggggctagactgctcaactgtggagcaattcattatactgaaaatgtgcttgttgttgaaaatttgtctgcatgttaatgcctcacccccaaacccttttctctctcactctctgcctccaacttcagattgactttcaatagtttttctaagacctttgaactgaatgttctcttcagccaaaacttggcgacttccacagaaaagtctgaccactgagaagaaggagagcagagatttaaccctttgtaaggccccatttggatccaggtctgctttctcatgtgtgagtcagggaggagctggagccagaggagaagaaaatgatagcttggctgttctcctgcttaggacactgactgaatagttaaactctcactgccactaccttttccccacctttaaaagacctgaatgaagttttctgccaaactccgtgaagccacaagcaccttatgtcctcccttcagtgttttgtgggcctgaatttcatcacactgcatttcagccatggtcatcaagcctgtttgcttcttttgggcatgttcacagattctctgttaagagcccccaccaccaagaaggttagcaggccaacagctctgacatctatctgtagatgccagtagtcacaaagatttcttaccaactctcagatcgctggagcccttagacaaactggaaagaaggcatcaaagggatcaggcaagctgggcgtcttgcccttgtcccccagagatgataccctcccagcaagtggagaagttctcacttccttctttagagcagctaaaggggctacccagatcagggttgaagagaaaactcaattaccagggtgggaagaatgaaggcactagaaccagaaaccctgcaaatgctcttcttgtcacccagcatatccacctgcagaagtcatgagaagagagaaggaacaaagaggagactctgactactgaattaaaatcttcagcggcaaagcctaaagccagatggacaccatctggtgagtttactcatcatcctcctctgctgctgattctgggctctgacattgcccatactcactcagattccccacctttgttgctgcctcttagtcagagggaggccaaaccattgagactttctacagaaccatggcttctttcggaaaggtctggttggtgtggctccaatactttgccacccatgaactcagggtgtgccctgggacactggttttatatagtcttttggcacacctgtgttctgttgacttcgttcttcaagcccaagtgcaagggaaaatgtccacctactttctcatcttggcctctgcctccttacttagctcttaatctcatctgttgaactcaagaaatcaagggccagtcatcaagctgcccattttaattgattcactctgtttgttgagaggatagtttctgagtgacatgatatgatccacaagggtttccttccctgatttctgcattgatattaatagccaaacgaacttcaaaacagctttaaataacaagggagaggggaacctaagatgagtaatatgccaatccaagactgctggagaaaactaaagctgacaggttccctttttggggtgggatagacatgttctggttttctttattattacacaatctggctcatgtacaggatcacttttagctgttttaaacagaaaaaaatatccaccactcttttcagttacactaggttacattttaataggtcctttacatctgttttggaatgattttcatcttttgtgatacacagattgaattatatcattttcatatctctccttgtaaatactagaagctctcctttacatttctctatcaaatttttcatctttatgggtttcccaattgtgactcttgtcttcatgaatatatgtttttcatttgcaaaagccaaaaatcagtgaaacagcagtgtaattaaaagcaacaactggattactccaaatttccaaatgacaaaactagggaaaaatagcctacacaagcctttaggcctactctttctgtgcttgggtttgagtgaacaaaggagattttagcttggctctgttctcccatggatgaaaggaggaggattttttttttcttttggccattgatgttctagccaatgtaattgacagaagtctcattttgcatgcgctctgctctacaaacagagttggtatggttggtatactgtactcacctgtgagggactggccactcagacccacttagctggtgagctagaagatgaggatcactcactggaaaagtcacaaggaccatctccaaacaagttggcagtgctcgatgtggacgaagagtgaggaagagaaaaagaaggagcaccagggagaaggctccgtctgtgctgggcagcagacagctgccaggatcacgaactctgtagtcaaagaaaagagtcgtgtggcagtttcagctctcgttcattgggcagctcgcctaggcccagcctctgagctgacatgggagttgttggattctttgtttcatagctttttctatgccataggcaatattgttgttcttggaaagtttattatttttttaactcccttactctgagaaagggatattttgaaggactgtcatatatctttgaaaaaagaaaatctgtaatacatatatttttatgtatgttcactggcactaaaaaatatagagagcttcattctgtcctttgggtagttgctgaggtaattgtccaggttgaaaaataatgtgctgatgctagagtccctctctgtccatactctacttctaaatacatataggcatacatagcaagttttatttgacttgtactttaagagaaaatatgtccaccatccacatgatgcacaaatgagctaacattgagcttcaagtagcttctaagtgtttgtttcattaggcacagcacagatgtggcctttccccccttctctcccttgatatctggcagggcataaaggcccaggccacttcctctgccccttcccagccctgcaccaaagctgcatttcaggagactctctccagacagcccagtaactacccgagcatggcccctgcatagccctggaaaaataagaggctgactgtctacgaattatcttgtgccagttgcccaggtgagagggcactgggccaagggagtggttttcatgtttgacccactacaaggggtcatgggaatcaggaatgccaaagcaccagatcaaatccaaaacttaaagtcaaaataagccattcagcatgttcagtttcttggaaaaggaagtttctacccctgatgcctttgtaggcagatctgttctcaccattaatctttttgaaaatcttttaaagcagtttttaaaaagagagatgaaagcatcacattatataaccaaagattacattgtacctgctaagataccaaaattcataagggcagggggggagcaagcattagtgcctctttgataagctgtccaaagacagactaaaggactctgctggtgactgacttataagagctttgtgggtttttttttccctaataatatacatgtttagaagaattgaaaataatttcgggaaaatgggattatgggtccttcactaagtgattttataagcagaactggctttccttttctctagtagttgctgagcaaattgttgaagctccatcattgcatggttggaaatggagctgttcttagccactgtgtttgctagtgcccatgttagcttatctgaagatgtgaaacccttgctgataagggagcatttaaagtactagattttgcactagagggacagcaggcagaaatccttatttctgcccactttggatggcacaaaaagttatctgcagttgaaggcagaaagttgaaatacattgtaaatgaatatttgtatccatgtttcaaaattgaaatatatatatatatatatatatatatatatatatatatatagtgtgtgtgtgtgttctgatagctttaactttctctgcatctttatatttggttccagatcacacctgatgccatgtacttgtgagagaggatgcagttttgttttggaagctctctcagaacaaacaagacacctggattgatcagttaactaaaagttttctcccctattgggtttgacccacaggtcctgtgaaggagcagagggataaaaagagtagaggacatgatacattgtactttactagttcaagacagatgaatgtggaaagcataaaaactcaatggaactgactgagatttaccacagggaaggcccaaacttggggccaaaagcctacccaagtgattgaccagtggccccctaatgggacctgagctgttggaagaagagaactgttccttggtcttcaccatccttgtgagagaagggcagtttcctgcattggaacctggagcaagcgctctatctttcacacaaattccctcacctgagattgaggtgctcttgttactgggtgtctgtgtgctgtaattctggttttggatatgttctgtaaagattttgacaaatgaaaatgtgtttttctctgttaaaacttgtcagagtactagaagttgtatctctgtaggtgcaggtccatttctgcccacaggtagggtgtttttctttgattaagagattgacacttctgttgcctaggacctcccaactcaaccatttctaggtgaaggcagaaaaatccacattagttactcctcttcagacatttcagctgagataacaaatcttttggaattttttcacccatagaaagagtggtagatatttgaatttagcaggtggagtttcatagtaaaaacagcttttgactcagctttgatttatcctcatttgatttggccagaaagtaggtaatatgcattgattggcttctgattccaattcagtatagcaaggtgctaggttttttcctttccccacctgtctcttagcctggggaattaaatgagaagccttagaatgggtggcccttgtgacctgaaacacttcccacataagctacttaacaagattgtcatggagctgcagattccattgcccaccaaagactagaacacacacatatccatacaccaaaggaaagacaattctgaaatgctgtttctctggtggttccctctctggctgctgcctcacagtatgggaacctgtactctgcagaggtgacaggccagatttgcattatctcacaaccttagcccttggtgctaactgtcctacagtgaagtgcctggggggttgtcctatcccataagccacttggatgctgacagcagccaccatcagaatgacccacgcaaaaaaaagaaaaaaaaaattaaaaagtcccctcacaacccagtgacacctttctgctttcctctagactggaacattgattagggagtgcctcagacatgacattcttgtgctgtccttggaattaatctggcagcaggagggagcagactatgtaaacagagataaaaattaattttcaatattgaaggaaaaaagaaataagaagagagagagaaagaaagcatcacacaaagattttcttaaaagaaacaattttgcttgaaatctctttagatggggctcatttctcacggtggcacttggcctccactgggcagcaggaccagctccaagcgctagtgttctgttctctttttgtaatcttggaatcttttgttgctctaaatacaattaaaaatggcagaaacttgtttgttggactacatgtgtgactttgggtctgtctctgcctctgctttcagaaatgtcatccattgtgtaaaatattggcttactggtctgccagctaaaacttggccacatcccctgttatggctgcaggatcgagttattgttaacaaagagacccaagaaaagctgctaatgtcctcttatcattgttgttaatttgttaaaacataaagaaatctaaaatttca

SEQ ID NO: 395 - DNA, 10257 bp, Homo sapiens
  source 1..10257: mol_type = other DNA
gcggagagaaccctctgttttcccccactctctctccacctcctcctgccttccccaccccgagtgcggagccagagatcaaaagatgaaaaggcagtcaggtcttcagtagccaaaaaacaaaacaaacaaaaacaaaaaagccgaaataaaagaaaaagataataactcagttcttatttgcacctacttcagtggacactgaatttggaaggtggaggattttgtttttttcttttaagatctgggcatcttttgaatctacccttcaagtattaagagacagactgtgagcctagcagggcagatcttgtccaccgtgtgtcttcttctgcacgagactttgaggctgtcagagcgctttttgcgtggttgctcccgcaagtttccttctctggagcttcccgcaggtgggcagctagctgcagcgactaccgcatcatcacagcctgttgaactcttctgagcaagagaaggggaggcggggtaagggaagtaggtggaagattcagccaagctcaaggatggaagtgcagttagggctgggaagggtctaccctcggccgccgtccaagacctaccgaggagctttccagaatctgttccagagcgtgcgcgaagtgatccagaacccgggccccaggcacccagaggccgcgagcgcagcacctcccggcgccagtttgctgctgctgcagcagcagcagcagcagcagcagcagcagcagcagcagcagcagcagcagcagcagcagcagcagcaagagactagccccaggcagcagcagcagcagcagggtgaggatggttctccccaagcccatcgtagaggccccacaggctacctggtcctggatgaggaacagcaaccttcacagccgcagtcggccctggagtgccaccccgagagaggttgcgtcccagagcctggagccgccgtggccgccagcaaggggctgccgcagcagctgccagcacctccggacgaggatgactcagctgccccatccacgttgtccctgctgggccccactttccccggcttaagcagctgctccgctgaccttaaagacatcctgagcgaggccagcaccatgcaactccttcagcaacagcagcaggaagcagtatccgaaggcagcagcagcgggagagcgagggaggcctcgggggctcccacttcctccaaggacaattacttagggggcacttcgaccatttctgacaacgccaaggagttgtgtaaggcagtgtcggtgtccatgggcctgggtgtggaggcgttggagcatctgagtccaggggaacagcttcggggggattgcatgtacgccccacttttgggagttccacccgctgtgcgtcccactccttgtgccccattggccgaatgcaaaggttctctgctagacgacagcgcaggcaagagcactgaagatactgctgagtattcccctttcaagggaggttacaccaaagggctagaaggcgagagcctaggctgctctggcagcgctgcagcagggagctccgggacacttgaactgccgtctaccctgtctctctacaagtccggagcactggacgaggcagctgcgtaccagagtcgcgactactacaactttccactggctctggccggaccgccgccccctccgccgcctccccatccccacgctcgcatcaagctggagaacccgctggactacggcagcgcctgggcggctgcggcggcgcagtgccgctatggggacctggcgagcctgcatggcgcgggtgcagcgggacccggttctgggtcaccctcagccgccgcttcctcatcctggcacactctcttcacagccgaagaaggccagttgtatggaccgtgtggtggtggtgggggtggtggcggcggcggcggcggcggcggcggcggcggcggcggcggcggcggcggcgaggcgggagctgtagccccctacggctacactcggccccctcaggggctggcgggccaggaaagcgacttcaccgcacctgatgtgtggtaccctggcggcatggtgagcagagtgccctatcccagtcccacttgtgtcaaaagcgaaatgggcccctggatggatagctactccggaccttacggggacatgcgtaggtgctgcgagcagagagggattcctcggaggtcatctgttccatcttcttgcctatgcaaatgcctgcctgaagctgctggaggctggctttgtaccggactttgtacagggaaccagggaaacgaatgcagagtgctcctgacattgcctgtcactttttcccatgatactctggcttcacagtttggagactgccagggaccatgttttgcccattgactattactttccaccccagaagacctgcctgatctgtggagatgaagcttctgggtgtcactatggagctctcacatgtggaagctgcaaggtcttcttcaaaagagccgctgaagggaaacagaagtacctgtgcgccagcagaaatgattgcactattgataaattccgaaggaaaaattgtccatcttgtcgtcttcggaaatgttatgaagcagggatgactctgggagcccggaagctgaagaaacttggtaatctgaaactacaggaggaaggagaggcttccagcaccaccagccccactgaggagacaacccagaagctgacagtgtcacacattgaaggctatgaatgtcagcccatctttctgaatgtcctggaagccattgagccaggtgtagtgtgtgctggacacgacaacaaccagcccgactcctttgcagccttgctctctagcctcaatgaactgggagagagacagcttgtacacgtggtcaagtgggccaaggccttgcctggcttccgcaacttacacgtggacgaccagatggctgtcattcagtactcctggatggggctcatggtgtttgccatgggctggcgatccttcaccaatgtcaactccaggatgctctacttcgcccctgatctggttttcaatgagtaccgcatgcacaagtcccggatgtacagccagtgtgtccgaatgaggcacctctctcaagagtttggatggctccaaatcaccccccaggaattcctgtgcatgaaagcactgctactcttcagcattattccagtggatgggctgaaaaatcaaaaattctttgatgaacttcgaatgaactacatcaaggaactcgatcgtatcattgcatgcaaaagaaaaaatcccacatcctgctcaagacgcttctaccagctcaccaagctcctggactccgtgcagcctattgcgagagagctgcatcagttcacttttgacctgctaatcaagtcacacatggtgagcgtggactttccggaaatgatggcagagatcatctctgtgcaagtgcccaagatcctttctgggaaagtcaagcccatctatttccacacccagtgaagcattggaaaccctatttccccaccccagctcatgccccctttcagatgtcttctgcctgttataactctgcactactcctctgcagtgccttggggaatttcctctattgatgtacagtctgtcatgaacatgttcctgaattctatttgctgggctttttttttctctttctctcctttctttttcttcttccctccctatctaaccctcccatggcaccttcagactttgcttcccattgtggctcctatctgtgttttgaatggtgttgtatgcctttaaatctgtgatgatcctcatatggcccagtgtcaagttgtgcttgtttacagcactactctgtgccagccacacaaacgtttacttatcttatgccacgggaagtttagagagctaagattatctggggaaatcaaaacaaaaacaagcaaacaaaaaaaaaaagcaaaaacaaaacaaaaaataagccaaaaaaccttgctagtgttttttcctcaaaaataaataaataaataaataaatacgtacatacatacacacatacatacaaacatatagaaatccccaaagaggccaatagtgacgagaaggtgaaaattgcaggcccatggggagttactgattttttcatctcctccctccacgggagactttattttctgccaatggctattgccattagagggcagagtgaccccagagctgagttgggcaggggggtggacagagaggagaggacaaggagggcaatggagcatcagtacctgcccacagccttggtccctgggggctagactgctcaactgtggagcaattcattatactgaaaatgtgcttgttgttgaaaatttgtctgcatgttaatgcctcacccccaaacccttttctctctcactctctgcctccaacttcagattgactttcaatagtttttctaagacctttgaactgaatgttctcttcagccaaaacttggcgacttccacagaaaagtctgaccactgagaagaaggagagcagagatttaaccctttgtaaggccccatttggatccaggtctgctttctcatgtgtgagtcagggaggagctggagccagaggagaagaaaatgatagcttggctgttctcctgcttaggacactgactgaatagttaaactctcactgccactaccttttccccacctttaaaagacctgaatgaagttttctgccaaactccgtgaagccacaagcaccttatgtcctcccttcagtgttttgtgggcctgaatttcatcacactgcatttcagccatggtcatcaagcctgtttgcttcttttgggcatgttcacagattctctgttaagagcccccaccaccaagaaggttagcaggccaacagctctgacatctatctgtagatgccagtagtcacaaagatttcttaccaactctcagatcgctggagcccttagacaaactggaaagaaggcatcaaagggatcaggcaagctgggcgtcttgcccttgtcccccagagatgataccctcccagcaagtggagaagttctcacttccttctttagagcagctaaaggggctacccagatcagggttgaagagaaaactcaattaccagggtgggaagaatgaaggcactagaaccagaaaccctgcaaatgctcttcttgtcacccagcatatccacctgcagaagtcatgagaagagagaaggaacaaagaggagactctgactactgaattaaaatcttcagcggcaaagcctaaagccagatggacaccatctggtgagtttactcatcatcctcctctgctgctgattctgggctctgacattgcccatactcactcagattccccacctttgttgctgcctcttagtcagagggaggccaaaccattgagactttctacagaaccatggcttctttcggaaaggtctggttggtgtggctccaatactttgccacccatgaactcagggtgtgccctgggacactggttttatatagtcttttggcacacctgtgttctgttgacttcgttcttcaagcccaagtgcaagggaaaatgtccacctactttctcatcttggcctctgcctccttacttagctcttaatctcatctgttgaactcaagaaatcaagggccagtcatcaagctgcccattttaattgattcactctgtttgttgagaggatagtttctgagtgacatgatatgatccacaagggtttccttccctgatttctgcattgatattaatagccaaacgaacttcaaaacagctttaaataacaagggagaggggaacctaagatgagtaatatgccaatccaagactgctggagaaaactaaagctgacaggttccctttttggggtgggatagacatgttctggttttctttattattacacaatctggctcatgtacaggatcacttttagctgttttaaacagaaaaaaatatccaccactcttttcagttacactaggttacattttaataggtcctttacatctgttttggaatgattttcatcttttgtgatacacagattgaattatatcattttcatatctctccttgtaaatactagaagctctcctttacatttctctatcaaatttttcatctttatgggtttcccaattgtgactcttgtcttcatgaatatatgtttttcatttgcaaaagccaaaaatcagtgaaacagcagtgtaattaaaagcaacaactggattactccaaatttccaaatgacaaaactagggaaaaatagcctacacaagcctttaggcctactctttctgtgcttgggtttgagtgaacaaaggagattttagcttggctctgttctcccatggatgaaaggaggaggattttttttttcttttggccattgatgttctagccaatgtaattgacagaagtctcattttgcatgcgctctgctctacaaacagagttggtatggttggtatactgtactcacctgtgagggactggccactcagacccacttagctggtgagctagaagatgaggatcactcactggaaaagtcacaaggaccatctccaaacaagttggcagtgctcgatgtggacgaagagtgaggaagagaaaaagaaggagcaccagggagaaggctccgtctgtgctgggcagcagacagctgccaggatcacgaactctgtagtcaaagaaaagagtcgtgtggcagtttcagctctcgttcattgggcagctcgcctaggcccagcctctgagctgacatgggagttgttggattctttgtttcatagctttttctatgccataggcaatattgttgttcttggaaagtttattatttttttaactcccttactctgagaaagggatattttgaaggactgtcatatatctttgaaaaaagaaaatctgtaatacatatatttttatgtatgttcactggcactaaaaaatatagagagcttcattctgtcctttgggtagttgctgaggtaattgtccaggttgaaaaataatgtgctgatgctagagtccctctctgtccatactctacttctaaatacatataggcatacatagcaagttttatttgacttgtactttaagagaaaatatgtccaccatccacatgatgcacaaatgagctaacattgagcttcaagtagcttctaagtgtttgtttcattaggcacagcacagatgtggcctttccccccttctctcccttgatatctggcagggcataaaggcccaggccacttcctctgccccttcccagccctgcaccaaagctgcatttcaggagactctctccagacagcccagtaactacccgagcatggcccctgcatagccctggaaaaataagaggctgactgtctacgaattatcttgtgccagttgcccaggtgagagggcactgggccaagggagtggttttcatgtttgacccactacaaggggtcatgggaatcaggaatgccaaagcaccagatcaaatccaaaacttaaagtcaaaataagccattcagcatgttcagtttcttggaaaaggaagtttctacccctgatgcctttgtaggcagatctgttctcaccattaatctttttgaaaatcttttaaagcagtttttaaaaagagagatgaaagcatcacattatataaccaaagattacattgtacctgctaagataccaaaattcataagggcagggggggagcaagcattagtgcctctttgataagctgtccaaagacagactaaaggactctgctggtgactgacttataagagctttgtgggtttttttttccctaataatatacatgtttagaagaattgaaaataatttcgggaaaatgggattatgggtccttcactaagtgattttataagcagaactggctttccttttctctagtagttgctgagcaaattgttgaagctccatcattgcatggttggaaatggagctgttcttagccactgtgtttgctagtgcccatgttagcttatctgaagatgtgaaacccttgctgataagggagcatttaaagtactagattttgcactagagggacagcaggcagaaatccttatttctgcccactttggatggcacaaaaagttatctgcagttgaaggcagaaagttgaaatacattgtaaatgaatatttgtatccatgtttcaaaattgaaatatatatatatatatatatatatatatatatatatatatagtgtgtgtgtgtgttctgatagctttaactttctctgcatctttatatttggttccagatcacacctgatgccatgtacttgtgagagaggatgcagttttgttttggaagctctctcagaacaaacaagacacctggattgatcagttaactaaaagttttctcccctattgggtttgacccacaggtcctgtgaaggagcagagggataaaaagagtagaggacatgatacattgtactttactagttcaagacagatgaatgtggaaagcataaaaactcaatggaactgactgagatttaccacagggaaggcccaaacttggggccaaaagcctacccaagtgattgaccagtggccccctaatgggacctgagctgttggaagaagagaactgttccttggtcttcaccatccttgtgagagaagggcagtttcctgcattggaacctggagcaagcgctctatctttcacacaaattccctcacctgagattgaggtgctcttgttactgggtgtctgtgtgctgtaattctggttttggatatgttctgtaaagattttgacaaatgaaaatgtgtttttctctgttaaaacttgtcagagtactagaagttgtatctctgtaggtgcaggtccatttctgcccacaggtagggtgtttttctttgattaagagattgacacttctgttgcctaggacctcccaactcaaccatttctaggtgaaggcagaaaaatccacattagttactcctcttcagacatttcagctgagataacaaatcttttggaattttttcacccatagaaagagtggtagatatttgaatttagcaggtggagtttcatagtaaaaacagcttttgactcagctttgatttatcctcatttgatttggccagaaagtaggtaatatgcattgattggcttctgattccaattcagtatagcaaggtgctaggttttttcctttccccacctgtctcttagcctggggaattaaatgagaagccttagaatgggtggcccttgtgacctgaaacacttcccacataagctacttaacaagattgtcatggagctgcagattccattgcccaccaaagactagaacacacacatatccatacaccaaaggaaagacaattctgaaatgctgtttctctggtggttccctctctggctgctgcctcacagtatgggaacctgtactctgcagaggtgacaggccagatttgcattatctcacaaccttagcccttggtgctaactgtcctacagtgaagtgcctggggggttgtcctatcccataagccacttggatgctgacagcagccaccatcagaatgacccacgcaaaaaaaagaaaaaaaaaattaaaaagtcccctcacaacccagtgacacctttctgctttcctctagactggaacattgattagggagtgcctcagacatgacattcttgtgctgtccttggaattaatctggcagcaggagggagcagactatgtaaacagagataaaaattaattttcaatattgaaggaaaaaagaaataagaagagagagagaaagaaagcatcacacaaagattttcttaaaagaaacaattttgcttgaaatctctttagatggggctcatttctcacggtggcacttggcctccactgggcagcaggaccagctccaagcgctagtgttctgttctctttttgtaatcttggaatcttttgttgctctaaatacaattaaaaatggcagaaacttgtttgttggactacatgtgtgactttgggtctgtctctgcctctgctttcagaaatgtcatccattgtgtaaaatattggcttactggtctgccagctaaaacttggccacatcccctgttatggctgcaggatcgagttattgttaacaaagagacccaagaaaagctgctaatgtcctcttatcattgttgttaatttgttaaaacataaagaaatctaaaatttcaaaaaa

SEQ ID NO: 396 - DNA, 10667 bp, Homo sapiens; identical to SEQ ID NO: 394
  source 1..10667: mol_type = other DNA

SEQ ID NO: 397 - protein, 11 aa, synthetic construct
SPKKKRKVEAS

SEQ ID NO: 398 - protein, 11 aa, synthetic construct
GPKKKRKVAAA

SEQ ID NO: 399 - protein, 7 aa, synthetic construct
PKKKRKV

SEQ ID NO: 400 - protein, 16 aa, synthetic construct
KRPAATKKAGQAKKKK

SEQ ID NO: 401 - protein, 9 aa, synthetic construct
PAAKRVKLD

SEQ ID NO: 402 - protein, 11 aa, synthetic construct
RQRRNELKRSP

SEQ ID NO: 403 - protein, 38 aa, synthetic construct
NQSSNFGPMKGGNFGGRSSGPYGGGGQYFAKPRNQGGY

SEQ ID NO: 404 - protein, 42 aa, synthetic construct
RMRIZFKNKGKDTAELRRRRVEVSVELRKAKKDEQILKRRNV

SEQ ID NO: 405 - protein, 8 aa, synthetic construct
VSRKRPRP

SEQ ID NO: 406 - protein, 8 aa, synthetic construct
PPKKARED

SEQ ID NO: 407 - protein, 8 aa, synthetic construct
POPKKKPL

SEQ ID NO: 408 - protein, 12 aa, synthetic construct
SALIKKKKKMAP

SEQ ID NO: 409 - protein, 5 aa, synthetic construct
DRLRR

SEQ ID NO: 410 - protein, 7 aa, synthetic construct
PKQKKRK